European Patent Specification EP 3 608 406 B1, published February 15, 2023. Title: COMPOSITIONS AND METHODS FOR MODULATING COMPLEMENT FACTOR B EXPRESSION. Applicant: Isis Pharmaceuticals. The sequence listing filed with the application follows.

SEQUENCE LISTING (854 sequences)

SEQ ID NO: 1 - DNA, 2646 bp, Homo sapiens
gacttctgcagtttctgtttccttgactggcagctcagcggggccctcccgcttggatgttccgggaaagtgatgtgggtaggacaggcggggcgagccgcaggtgccagaacacagattgtataaaaggctgggggctggtggggagcaggggaagggaatgtgaccaggtctaggtctggagtttcagcttggacactgagccaagcagacaagcaaagcaagccaggacacaccatcctgccccaggcccagcttctctcctgccttccaacgccatggggagcaatctcagcccccaactctgcctgatgccctttatcttgggcctcttgtctggaggtgtgaccaccactccatggtctttggcccggccccagggatcctgctctctggagggggtagagatcaaaggcggctccttccgacttctccaagagggccaggcactggagtacgtgtgtccttctggcttctacccgtaccctgtgcagacacgtacctgcagatctacggggtcctggagcaccctgaagactcaagaccaaaagactgtcaggaaggcagagtgcagagcaatccactgtccaagaccacacgacttcgagaacggggaatactggccccggtctccctactacaatgtgagtgatgagatctctttccactgctatgacggttacactctccggggctctgccaatcgcacctgccaagtgaatggccgatggagtgggcagacagcgatctgtgacaacggagcggggtactgctccaacccgggcatccccattggcacaaggaaggtgggcagccagtaccgccttgaagacagcgtcacctaccactgcagccgggggcttaccctgcgtggctcccagcggcgaacgtgtcaggaaggtggctcttggagcgggacggagccttcctgccaagactccttcatgtacgacacccctcaagaggtggccgaagctttcctgtcttccctgacagagaccatagaaggagtcgatgctgaggatgggcacggcccaggggaacaacagaagcggaagatcgtcctggacccttcaggctccatgaacatctacctggtgctagatggatcagacagcattggggccagcaacttcacaggagccaaaaagtgtctagtcaacttaattgagaaggtggcaagttatggtgtgaagccaagatatggtctagtgacatatgccacataccccaaaatttgggtcaaagtgtctgaagcagacagcagtaatgcagactgggtcacgaagcagctcaatgaaatcaattatgaagaccacaagttgaagtcagggactaacaccaagaaggccctccaggcagtgtacagcatgatgagctggccagatgacgtccctcctgaaggctggaaccgcacccgccatgtcatcatcctcatgactgatggattgcacaacatgggcggggacccaattactgtcattgatgagatccgggacttgctatacattggcaaggatcgcaaaaacccaagggaggattatctggatgtctatgtgtttggggtcgggcctttggtgaaccaagtgaacatcaatgctttggcttccaagaaagacaatgagcaacatgtgttcaaagtcaaggatatggaaaacctggaagatgttttctaccaaatgatcgatgaaagccagtctctgagtctctgtggcatggtttgggaacacaggaagggtaccgattaccacaagcaaccatggcaggccaagatctcagtcattcgcccttcaaagggacacgagagctgtatgggggctgtggtgtctgagtactttgtgctgacagcagcacattgtttcactgtggatgacaaggaacactcaatcaaggtcagcgtaggaggggagaagcgggacctggagatagaagtagtcctatttcaccccaactacaacattaatgggaaaaaagaagcaggaattcctgaattttatgactatgacgttgccctgatcaagctcaagaataagctgaaatatggccagactatcaggcccatttgtctcccctgcaccgagggaacaactcgagctttgaggcttcctccaactaccacttgccagcaacaaaaggaagagctgctccctgcacaggatatcaaagctctgtttgtgtctgaggaggagaaaaagctgactcggaaggaggtctacatcaagaatggggataagaaaggcagctgtgagagagatgctcaatatgccccaggctatgacaaagtcaaggacatctcagaggtggtcacccctcggttcctttgtactggaggagtgagtccctatgctgaccccaatacttgcagaggtgattctggcggccccttgatagttcacaagagaagtcgtttcattcaagttggtgtaatcagctggggagtagtggatgtctgcaaaaaccagaagcggcaaaagcaggtacctgctcacgcccgagactttcacatcaacctctttcaagtgctgccctggctgaaggagaaactccaagatgaggatttgggttttctataaggggtttcctgctggacaggggcgtgggattgaattaaaacagctgcgacaacaaaaaaaaaaaaaaaaaaaa

SEQ ID NO: 2 - DNA, 9001 bp, Homo sapiens
ggaggtgagggtctcaggttggggatgctgggatccccctgtgacagctcccagaatgtctctcttccttctccaggtctggctgctttctctctctgacgcgggtcacccctcctcccaagcctcacaaacctgctaggtgtccctgggtctgcttattctttttttgttgttattgagatggagtcttgctctgtctcccaggctggagtgcagtggcacgacctcagctcactgcaacttctgcctcctgggttcaagcgattctcctacttcagcctcccgagtagctgagattacaggtgcccaccaccacaccagctaatttttgtatttttagtagagacgggatttcgccatgttggccaggatggtcttgaactcctgacctcaagtgatctgcctgcctcaacctcccaaagtgctgagattacaggcgtgagccactgcacccacccgggtctgcttattctacccttctctctggttccacccctgctgcagtggacaagctgtgccgaggttgtctcccaagaaaaaaccatgttccccaacttgacagatgtcagggaggtggtgacagaccagttcctatgcagtgggacccaggaggatgagagtccctgcaagggtgagtccctcaccatgcctggattcccaaggggaaggccacctgtgtctctgtggccagcatgcatgccagaacaccagtccactgccctagatgacactgtctcctgtcaccctttgctggcaggagaatctgggggagcagttttccttgagcggagattcaggttttttcaggtgagaaggtagaagcttgcaggacccaggggttacaggatctcagccttgttggggggatgagggaggcctttgagggatctagggaggttggggcttacagttggggctgtggcagcctcccagccagttctctccttttctccaggtgggtctggtgagctggggtctttacaacccctgccttggctctgctgacaaaaactcccgcaaaagggcccctcgtagcaaggtcccgccgccacgagactttcacatcaatctcttccgcatgcagccctggctgaggcagcacctgggggatgtcctgaattttttacccctctagccatggccactgagccctctgctgccctgccagaatctgccgcccctccatcttctacctctgaatggccacccttagaccctgtgatccatcctctctcctagctgagtaaatccgggtctctaggatgccagaggcagcgcacacaagctgggaaatcctcagggctcctaccagcaggactgcctcgctgccccacctcccgctccttggcctgtccccagattccttccctggttgacttgactcatgcttgtttcactttcacatggaatttcccagttatgaaattaataaaaatcaatggtttccacatctctcagtgcctctatctggaggccaggtagggctggccttgggggagggggaggccagaatgactccaagagctacaggaaggcaggtcagagaccccactggacaaacagtggctggactctgcaccataacacacaatcaacaggggagtgagctggatccttatttctggtccctaagtgggtggtttgggcttactggggaggagctaaggccggagaggaggtactgaaggggagagtcctggacctttggcagcaaagggtgggacttctgcagtttctgtttccttgactggcagctcagcggggccctcccgcttggatgttccgggaaagtgatgtgggtaggacaggcggggcgagccgcaggtgccagaacacagattgtataaaaggctgggggctggtggggagcaggggaagggaatgtgaccaggtctaggtctggagtttcagcttggacactgagccaagcagacaagcaaagcaagccaggacacaccatcctgccccaggcccagcttctctcctgccttccaacgccatggggagcaatctcagcccccaactctgcctgatgccctttatcttgggcctcttgtctggaggtaagcgagggtaaccttcccttcctgctgtctccagcatccctccttggccttttggggccaggcttcatcagcctttctcttcaggtgtgaccaccactccatggtctttggcccggccccagggatcctgctctctggagggggtagagatcaaaggcggctccttccgacttctccaagagggccaggcactggagtacgtgtgtccttctggcttctacccgtaccctgtgcagacacgtacctgcagatctacggggtcctggagcaccctgaagactcaagaccaaaagactgtcaggaaggcagagtgcagaggtttgagggcaatgagtgtgggcagtggcctaaggcagaaacagggcaggcggcagcaaggtcaggactaggatgagactaggcagggtgacaaggtgggctgaccgggagtaggagcagttttagggtggcaggcggaaagggggcaagaaaaagcggagttaacccttactaagcatttaccctgggcttccaggcagccctggaagtcaagagaacactcagaaatggggagggagaagcagtggaaatccatatgggttgaggagtaggtaagatgctgcttctgcgggactgggaatgcgctgtttctcagtgacatggtctccgagaccaggagggatacacctaaggcagcctttccctcttgatgacttctacttgtccccccttctcaaagcaatccactgtccaagaccacacgacttcgagaacggggaatactggccccggtctccctactacaatgtgagtgatgagatctctttccactgctatgacggttacactctccggggctctgccaatcgcacctgccaagtgaatggccgatggagtgggcagacagcgatctgtgacaacggaggtgagaagcatcccctccccctacattgctgtctccctgacggcgcccagcccgaggagtgggcactcggctccggacactgtaactcttgctctctaccttgctcacggggcctcaggcttcagtgcttacctcgatgtctcatacctctgcagcggggtactgctccaacccgggcatccccattggcacaaggaaggtgggcagccagtaccgccttgaagacagcgtcacctaccactgcagccgggggcttaccctgcgtggctcccagcggcgaacgtgtcaggaaggtggctcttggagcgggacggagccttcctgccaaggtgacctttgacctgtacccccaggtcagatcctggtcttccatcctactgtcttctctccccacctcaaccctgctctttcctcactttgtttaaacctccctgtacaactatctcacttctgagccttttataccctggaaacccatgatcccccgtctctttggtcactgtatccctgacactcccagacatttgacctcatttctgactctcccagactccttcatgtacgacacccctcaagaggtggccgaagctttcctgtcttccctgacagagaccatagaaggagtcgatgctgaggatgggcacggcccaggtttgaagacagagaagggaggcagggcagggaactgggggaaaatggagaagggacagaactgttaatgctggagcctgagccactctcctggcacccaggggaacaacagaagcggaagatcgtcctggacccttcaggctccatgaacatctacctggtgctagatggatcagacagcattggggccagcaacttcacaggagccaaaaagtgtctagtcaacttaattgagaaggtggaatcctcctatccctgaactcgggggaatggaatctcgctgatcttccaggactagctccctgatcattccagcccctctgaacaacagggccccaggaaaatctccaggtcctattctgtcctccttcccttttacttgaagcagtttcttgactggtaattcctccatgaacctcagcccttgagcctcttactgagagcctccctgtcccagcaaagtcgctgaaatctcccaatcacagtattctattttcaatgccatggcgccttgttctcctcacccacaggtggcaagttatggtgtgaagccaagatatggtctagtgacatatgccacataccccaaaatttgggtcaaagtgtctgaagcagacagcagtaatgcagactgggtcacgaagcagctcaatgaaatcaattatgaaggtcagaggttagggaatggtgggaggttcactttggggtcaggaggttcagggtggagggggtcatgagactaccttgagggcgacagggaggaccactttgtagtcaaaagttgaacagcaggatcgttgggcaatggaggttagtgggaacctgttgggggctggaagggccactttgtggtcaaagggaagtccgtgtaatgatgattaacttaaaaagttgaaagatgtgggatttcagttgcagattggtctctggggttaaaagatggcttggaagaccaggtgaggtgatggtctcttccctctccacagaccacaagttgaagtcagggactaacaccaagaaggccctccaggcagtgtacagcatgatgagctggccagatgacgtccctcctgaaggctggaaccgcacccgccatgtcatcatcctcatgactgatggtcagaagggacctctctcctgtcccagcctccccaccttctcagaccagcatgtggcccttaagtccacttgtaacactatacccatggttggggccctgaatgtgactcatagctggctgttcatctctcctgtgacccttcataaggaattcttcctaagccctgtgatcaactatctctaacccttcctcaacttgctcaccctgccatgtgtatccctgcctttagccagtttatcttccttatctcctaccctcatggtcctgtctcttctgcaggattgcacaacatgggcggggacccaattactgtcattgatgagatccgggacttgctatacattggcaaggatcgcaaaaacccaagggaggattatctgggtgagtaacctgcctaggacccagcaccccacttcctcagggcttggaccctcatccttcctttttatccctcagatgtctatgtgtttggggtcgggcctttggtgaaccaagtgaacatcaatgctttggcttccaagaaagacaatgagcaacatgtgttcaaagtcaaggatatggaaaacctggaagatgttttctaccaaatgatcggtagggagatacaagggaataaagaacacaactctcctcaggttcccctgaagtaattcattcttcctctacacctgaagctctagttgcctggaaagccttcttcattcctccttctctacctcagtgtcactattcttgtttcctggcactgttcacttaaccttagaatcacagagctctgagcacttcagagatctttctatagtcctacatttgacacgtggaaacagaagccaaaggaggtcaagggacagcaagttagcaacaagggtgggcttgaaaacagccaggcctctgacagcttgatcccaagttctttcccttttcagtccaccatagcagttttctcctaacacgaggaaacaaatacccgtggtctttccctttctccttttgggcctttgctccccatagactcctacccaaaaggctgctgccatttgggaatgaagtgttccgagttttcagcacattctccttctctgccagatgaaagccagtctctgagtctctgtggcatggtttgggaacacaggaagggtaccgattaccacaagcaaccatggcaggccaagatctcagtcattgtaagcacagaatcccagtagtggggacttgggggaggtgaggtcaaggtgaaatgggagtaggggaaggaaaaaatggccataagagatggtggtttgtgaaagttgagctttccctctctactgttgtgtccccagcgcccttcaaagggacacgagagctgtatgggggctgtggtgtctgagtactttgtgctgacagcagcacattgtttcactgtggatgacaaggaacactcaatcaaggtcagcgtaggtaaggatgcaactgaaggtcctgggctgcacctatgctctccaggcaacacctcccactttctacagatcctacactccacccatcctcaatgcagccccattccttgcaccccagaccagtcagggatgggggaagacgtgaagttaggaatgacacggggccagaggcaggaagctgcccacaaagaggtggtacctactctcctacttcaggaggggagaagcgggacctggagatagaagtagtcctatttcaccccaactacaacattaatgggaaaaaagaagcaggaattcctgaattttatgactatgacgttgccctgatcaagctcaagaataagctgaaatatggccagactatcaggtgagagcgtccagatccctgaggaaaggctgggaaaggctggaggactggggtgaggagcaggcctggtttgctgttctccttgtcctttataggcccatttgtctcccctgcaccgagggaacaactcgagctttgaggcttcctccaactaccacttgccagcaacaaagtaagacatacttggcaagaggataaggatgagatcccaagagacaagtggggcatgagagggaggtgcaataggaagagatgatgcctggcccagaacctagctctagaagggcttaggggacatctactgagtgacaaaggcaatggggagatgacagtggtgggagcagctgaagtgacgcagtctattcgtccagaggaagagctgctccctgcacaggatatcaaagctctgtttgtgtctgaggaggagaaaaagctgactcggaaggaggtctacatcaagaatggggataaggtgagaaacgggcatcctaaggaggcactctaggccccaatccttcctaagccacttctgttcattacttctccatgcttcccacctcccctacagaaaggcagctgtgagagagatgctcaatatgccccaggctatgacaaagtcaaggacatctcagaggtggtcacccctcggttcctttgtactggaggagtgagtccctatgctgaccccaatacttgcagaggtgagagaatgctctttggttgtgctacaagtgcccaaggcccaacagtccttttctctacagcttctcctctccttgcaggtgattctggcggccccttgatagttcacaagagaagtcgtttcattcaagtgagtcctccctttcctatctggggagatgccaagtggtcagcatgggccccaaagcaggaaagctcaatgcatgtggctagtaattcgaggtaggcagagcctgcctcaccttaggaccgcatgtcttgcctgcgtgtgtcaagaacgaggctgagctgggtccctagtctgattcctttaggtcagctaagacacaagcaggaacagccatgcttccaggattaggaattctactgaatgatccatggcaccccactgcctctgcaggttggtgtaatcagctggggagtagtggatgtctgcaaaaaccagaagcggcaaaagcaggtacctgctcacgcccgagactttcacatcaacctctttcaagtgctgccctggctgaaggagaaactccaagatgaggatttgggttttctataaggggtttcctgctggacaggggcgtgggattgaattaaaacagctgcgacaacacctgtgttccagatccttttggggcaagggagtggggaacaggcactggccatgttgttacactgagatcaaacctgacagccgtttttaaaggtttaaccccaatcccaagtgctgaaaaaccagaggctgagggagatgtgtaagcttccacctcagtgttttactgagaccagcattggggcatatgaggcacaaggaatccagctctgttccctagaagccatccacaaggttttccttgtagacgtcatcactgtagacaatctgggtcctcttgtcccggtggcaacccttagggctgttctggacagctagggagggaggagaggaacagttaaggtctaaaggagatcatagaacagaccctgaggctgactcctgaccacctcactcctggccactggcccctggaagcccagtttccacgctgccctctggtggccaggatggcctgtcttccttagctcctttgtgccaacccatggccaagaaaagtataagtggacattttgatgaatgttttgttcttagaaaaatcccaaatgtcattgttgagacacgtgaatgatattaacccactacttacagtcagtatgtcagaagctaaaaactagaaaacctctgtagcccttttttgacatgctggtcaattctagttcctttcttttgcctgaagggccactgtagctgagcccttctttctgctcactcctttcccaggaaaatctactttcagggaaaatggattattcacactaagaaatgctactagctccaccagaactcattcagggtgtagctttggccctcaccattctctctcaagcctctagctgtttcttccccttcctctttcctccctccaccagacatgttactctcttcaccccatccaatggttccatccccaccacccttgagctacagagaatctctctcacccactcccatcctgtgatctctgtgcctcaacactgctggctactccctctttctcaaagtgtgtgtccttttgcttcagtggcccaggcccctgcggtgctgctcccagccctccgacccctcctcctgtctcctttgctaacgttaggctcaacgttagcctaacatgtcaggacagctggggacatgtgggg

SEQ ID NO: 3 - DNA, 9001 bp, Macaca mulatta
gatggaatcttgctctgtctcccacactggagtgcagtggcacgatcttggctcactgcgacttctgcctcccagatttaagtgattctcctacctcggcctcccaagtagctgggattataggtgcttgccaccacatgcagctaatttttgtatttttagtagagacaggattccgccatgttggccaggatggtcttgaactcctgacctcaagtgattcgcccacctcagcctcccaaactgctgggattacaggcgtgagccattgcacccagtcaggtctgcttattcttcccttctctctggttccacccctacggcagtggacaagctgtgccgaggtcgtctcccaagaaaaaaccatgttccccaacttgacagatgtcagggaggtggtgacagaccagtttctatgcagtgggacccaggaggatgagagtccctgcaagggtgagtccctcaccatgcctggattcccaaaggggaaggccacctgtgtctctgtggccagggtgcatgccagaacaccagtccactgccctgtatgacgctgtctcctgtcaccctttgctggcaggagaatctgggggagcagttttccttgagcggagattcaggttttttcaggtgagaaggtggaagcttgcaggacccaggggttacaggatgtcagccttgttggggggatgagggaggcctttgagggatctagggaggttggggcttacagctggagctgtggcagcctcccagccagttctctccttttctccaggtgggtctggtgagctggggtctttacaacccctgccttggctctgctgacaaaaactcccgcaaaagggcccctcgtagcaaggtcccgccgccacgagactttcacatcaatctcttccgcatgcagccctggctgaggcagcacctgggggatgtcctgaattttttacccctttagtcatggccactgagccctctgctgtcctgttagaatccgccccccctccatcttctacctctgaatgcccacccttagactctgtgacccatgctgtctcctagttgagtaaatctgggtctctaggatgccaggggcagcgcacacaagctgggaaatcctcagggctcctaccagcgggactgcctcgctgccccacctcccgctccttggcctgtccccaaattcctcccctggttgacttgactcatgctcatttcactttcatatggaatttcccagttatgaaattaataaaaatcagtggtttccacatctgtctgtgactctatctggaggccaggtagggctggcctggggggaaggggaggccagaatgactccaagagccacaggaaggcaggtcagagaccccactggacaaacagtggctggactctgtaccataacacacaagcaacaggggagtgagctggatccttatttctggtccctaagtgggtggtctgggcttgctggggaggagctgaggccagaaggaggtactgaaggggagagtcctggaccttgggcagcaaagggtgggacttctgcagtttctgcttccttgactggcagctcagcggggccctcccgcttggatgttccgggaaagtgatgagggtaggacaggcggggcaagctgcaggtgccagaacacagattgcataaaaggccgggagctggtggggggcaggggaagggaatgtgaccaggtctaggtctggagtttcagcttggacactgagctaagtagacaagcaaaacaagccaggacacgccatcctgccccaggcccagcttctctcctgccttctaacgccatggggagcagtctcagcccccagctctacctgatgcccttcatcttgggcctcttatctggaggtaagtgagggtaaccttcccttcctgctgtccccagcatccctccttggccttttggggccaggcttcatcagcctttctcttcaggtgtgaccaccactccattgtcttcggcccagcctcaaggatcctgctctctggagggggtagagatcaaaggtggctccttccgacttctccaagagggccaggcactggaatacgtgtgtccttctggcttctacccgtaccctgtgcagacacgtacctgcagatccacggggtcctggagcaccctgcagactcaagatcgaaaaactgtcaagaaggcagagtgcagaggtttgagggcaatgagtgtgggcagtggcctaagggagaaacagggcagatggcagcaaggtcaggactaggatgagactaggcagggtgacaaggtgggctgaccaggagtaggagcagttttagggttgtagagggaaaggaagggaaaaaaaaaggggagttaacctttagtaagcatttaccctgggcttccacgcagccctggaagtcaagagaacactcagcaatggggagggaggagcagcggaaacccctatgggttgaagggtaggtaagatgcagcttctgcaggactgggaatgctctgtttctcagtgacctggtctctgagaccaggagggaaacacctaaggcagcctttccctcttaatgacttctacttctcccctcttctcaaagcaatccgctgtccacgaccacaggacttcgagaacggggaataccggccccggtctccctactacaatgtgagtgatgagatctctttccactgctatgacggttacactctccggggctctgccaatcgcacctgccaagtgaatggccggtggagtgggcagacagcgatctgtgacaacggaggtgagaagcatcctctccccccacattgctgtctccctgacagcgcctagcctgaggagtgggcatttgcccccggacactgtaactcttgctctctaccttgccctcggggcctcaggcttcagcgcttacctccatgtctcatgcctctgcagcggggtactgctccaacccaggcatccccattggcacaaggaaggtgggcagccggtaccgccttgaagacagcgtcacctaccactgcagccgggggcttaccctgcgtggctcccagcggcgaacatgtcaggaaggtggctcttggagcgggacggagccttcctgccaaggtgacccttgacctgtacccccaggtcagatcctgatcttgcatcctactgtcttctctccccacctcaaccctgctctttcctcacttcttttaaaccttcctctagaactgtctcacttctgagccttttctaccctggaaacccacaatcccctgtctctttggtcactgtgtccctgacactcccagacatttgacctcatttctgactctcccagactccttcatgtacgacacccctcaagaggtggccgaagctttcctgtcttccctgacggagaccatagaaggagtcgatgccgaggatgggcacagcccaggtttgaaggcagagaggggaggcaaggcagggaactgggggaaaatggagaagggacaagataatcgttcatgctggagcctgagtcactctcctggcacccaggggaacaacagaagcggaggatcatcctagacccttcaggctccatgaacatctacctggtgctagatggatcagacagcattggggccggcaacttcacaggagccaaaaagtgtctagtcaacttaattgagaaggtggagtcctcctatccctgaacttgggggaatggaatcttgctgatcttccaggactagctccctgatcattccagcccctctgaaccgcagggccccaggaaagtctccaggtcctattctgtcctccttcccttgtacttgattcctccatgaacctgtgcttgagcctcttcctaagagcctccctgtcccagcaacgttgctgaagtctcccaatcacagtattctactttcaatgccatggcgccttgttctcctcacccacaggtggcaagttatggtgtgaagccaagatatgctctagtgacatatgccacataccccagaatttgggtcaaagtgtctgaccaagagagcagcaatgcagactgggtcacgaagaagctcagtgaaatcaattatgaaggtcagaggttagggaatggtgggaggttcactttggggtcaggaggttcaggagtgttgtgtggagggggtcatgagactaccttgagggcaacagggggaccactttgtagtcaaaggttgaacagcaggatcattgggcaatggaggttagtgggaacctgctgagggctggaagggccactttgtggtcaaagggaagtccatatgatgattaacttaaaaagttgaagatgtgagatttcagttgcagattggtctctggggttaaaagatggcttggaagaccaggtgaggcgatgctctcttccctccccacagaccacaagttgaagtcagggactaacaccaagagggccctccaggcagtgtacagcatgatgagttggccagaggacatccctcctgaaggctggaaccgcacccgccatgtcatcatcctcatgaccgatggtcagaagggacctctctcctgtcccagcctccccaccttctcagaccagcatgtggcccttaagtccacttgtaacactatacccatggttggggccctgaatgtgactcgtaactggctgttcatctctcctgtgacccttcataaagaattattcctaaagccctgtgatcaactacctctaacccttcctcaacttactcaccctgccacgtgtatcactgcctctagccaatttatcttatctcctaccctcatggtcccgtctcttctgcaggattgcacaacatgggcggggacccaattactgtcattgatgagatccgggacttgttatacatcggcaaggatcgtaaaaacccgagggaggattatctgggtgagtaacctgcctaggacccagcaccctacttcctcagggcttggaccgtcatccttcctttttctccctcagatgtctatgtgtttggggttggacctttggtggaccaagtgaacatcaatgctttggcttccaagaaagacaatgagcaacatgtgttcaaagtcaaggatatggaaaacctggaagacgttttcttccaaatgattggtaggcagacacaagggaatcaagaacgcaactctcctcagcttcccctgaaataattcattcttcctctacccctgaagctctagttgcctggaaagccttcttcattcctccttctctacctcagtatcactattcttgtttcctggcactgtttgcttcttaaccttagaatcacagagctctaggcacttcagagatctttctattgtcctacatttgacacatgtggaaacaaaggccaaaggaggtcaaggggcagcaagctagcaacagggctgggcttgaaaacagccaggcctctgatagcttgatcccaagttctttcccttttcactccaccacagcagttttctcctaacacgaggaaacaaatacctgtggcctttccctttctccttttgggcctctgccccccacagacttctacccaaaggctgctgccgtttgggaatgaagtgttccaagttttcagcacattctccttctctgccagatgaaagccagtctctgagtctctgtggcatggtttgggaacacagcaagggtaccgattaccacaagcaaccatggcaggccaagatctcagtcactgtaagcacagaatcccagtagtgaggacttgggggaggtgaggtcaaggtgaaatgggagtaggggaagggcaaaatggccgtaagagatggtggtttgtgaaagttgagttttccctttctactgttctgttcccagcgcccttcgaagggacatgagagctgtatgggggctgtggtgtctgagtactttgtgctgacagcagcacattgttttactgtggacgacaaggaacactcaatcaaggtcagcgtgggtaaggatgcaactgaaggtcccgggctgcacctacgccctccaggcaacacctcccactttctacagatcccacactccactcatctgcaatgcagccccatcccttgcaccccagaccagtcagggatggggaagacttgaagttaggaatgacatggggccagaggcaagaagctgcccacaaagaggtggtacctattctcctacttcaagggaagaagcgggacctggagatagaaaaagtcctatttcaccccgactacaacattagcgagaaaaaagaagcaggaattcctgaattttatgactatgacgttgccctgatcaagctcaagaataagttgaattatgacccgactatcaggtgagagcatccagatccctgaggaaaggctgggaaaggctggaggactggggtgaggagcaggcctagtttgctgttctttctccatcctttataggcccatttgtctcccctgcaccgagggaacaactcgagctttgaggcttcctccaactaccacttgccagcaacagagtaagacatactaggggggaggataaggatgagatcccgagacaagtgaggcatgagagggagatgcaataggaagagacgatgcctggcccagaacctagcactaggaagggcttaggggacatctgctgagtgacaaagtcaatagggagatgacagtggtgggagcagctgaagtgatgcagtctatttgtccagaggaagagctgctccctgcacaggatatcaaagctctgtttgtgtctgaggaggagaagaagctgactcggaaggaggtctacatcaagaatggggataaggtgagaaatgggcatcctaaggaggcactctaggccctaatccttcctaagccacctctgttcattacctttctccatgcttcccacctcccctacagaaaggcagctgtgagagagatgctcaatatgccccaggctatgacaaagtcaaggacatctcggaggtggtcacccctcggttcctttgtactggaggagtgagtccctatgctgaccccaatacttgcagaggtgagagaacgctctctggttgtgctccaagtgcccgagggccaagagtccttttccctacagcttctcctctccttgcaggtgattctggcggccccttgatagttcacaagagaagtcgtttcattcaagtgagtcctccctttcctatctggggagatgccaagtggtcagcatgggccccaaagcaggaaagcacaatgcatgtggctagtaattcgaggtgggcagagcctgcctcactttaggactgcatgtctggcctgtgtgtgtcaagaatgaggctgagctgggtccctagcctgattcctttaggtcagctaagacacaatcaggaacagtcatgcttccaggattaggaattctatgaatgatccatggcaccccactgcctctgcaggttggtgtcatcagctggggagtagtggatgtctgcaaaaaccagaagcggcaaaagcaggtacctgctcacgcccgagactttcacgtcaacctcttccaagtgctgccctggctgaaggagaaactccaagatgaggatttgggttttctctaaggggtttcctgctggacaggggcgcgggattgaattaaaacagctgcgacaacacttgtgttccagatccttttggggcaagggagtggggaacgggcactggccatgttgttacactgagatcaaacctgacacccatttttaaaggcttaaccccaatcccaagtgctgaaaaaccagaggctgagggagatatgtaagcttccacctcagtgttttactgagaccagcattggggcatttgaggcacaaggaatccagctctgttccctagaagccatccacaaggttttccttgtagacgtcatcactgtagacaatctgggtcctcttgtcccggtggcaacccttagggctgttctggacagctagggagggaggagaggaacagttaaggtctaaaggagatcatagatcagaccctgaggctgactcctgaccacctcagtcctggctgctggcccctggaaacccagtttccacgctgccctctggtggccaggatggcctgtcttccttagctcctttgtgccaacccatggccaaggagagtgtaagtggacattttgatgaatgttttgttcttagaaaaatcccaaatgtcattgttgagatatatgaatgatattaacccactacttatagtcagtatgtcagaagctaaaaactagaaaacctctgtagccctttattgacatgctggtcaactctagttcctttcttttgcctgaaaggccactgttgctctgagtccttctttctgctcactcctttcccaggaaaatctactttcaggtaaatgggttactcatactaaggaatgctactagctccaccagaactcatccagcatgtagctttggccctcaccattctctctcaagcctctagctgtttcttccccttcctcttttcctccctccaccagacatgttactctcttcaccccatccaaagattccatccccaccacccttgacctagagagaatctctcccacccacttctcatcctgtgatctctgtaccttgacactgctggctactccctctttctcaaagcatgtgtcctttcgcttcagtggcccaggcccctctggtgctgctcccagccctctgacccctcctcctgtctcctttgctaacgttaggctcaacgttagcctaacgtgtcaggagagctggagacacgtggggcgtaaggtggacagtcctgtttcctaacatagtccctgagtattcctcaagtctagtcctgggtcgttttttttctccgaaatcagtctccctcatgatcggggagccaccctgtgatgcagatgacttaatctatgttttcattccttacctcacacctgagttccagacccctaatttcaaatactt

SEQ ID NO: 4 - DNA, 4086 bp, Macaca mulatta
atagatatattagcatcagggagacagggcaaaggttccacccttcagctcagtccccagtccctgcttattatttccctaacagaagaccatcccccttgccactccctgggttttcttctctggcagcaatgaagcagctgctgagccagctctggttttcgggaagtcagatgaccttttccctcccgcggctctctgcctctcgctgtccctagggaggacaccatggacccactgatggttcttttttgcctgctgttcctgtacccaggtccggcagactcggctacctcctgccctcagaacgtgaatatctctggtggcaccttcaccctcagccatggctgggcccctgggagccttctcatctactcctgtccccagggcctgtacccatccccagcgtcacggctgtgcaagagcagcggacagtggcagaccccaagagccacccggtctctgactaaggcggtctgcaaacctggccactgccccaaccccggcatttcgctgggcgcggtgcggacaggctcccgctttggtcatggggacaaggtccgctatcgctgctcctcgaatcttgtgctcacggggtctgcggagcgggagtgccagggcaacggggtctggagtggaacggagcccatctgccgccagccctactcttatgacttccctgaggacgtggcccctgccctgggcacctccttctcccacatgcttggggccaccaatcccacccagaggacaaaggatcatgaaaatggaactgggactaacacctatgcagccctaaacagtgtctatctcatgatgaacaatcaaatgcaactccttggcatgaaaacgatggcctggcaggaaatccgacatgccatcatccttctgacagatggaaagtccaatatgggtggctctcccaaaacagctgttgaccaaatcagagagatcttgaatatcaaccagaagaggaatgactatctggacatctatgccatcggggtgggcaagctggatgtggactggagagaactgaatgagctggggtccaagaaggatggcgagaggcatgccttcattctgcaggacacaaaggctctgcaccaggtctttgaacatatgctggatgtctccaagctcacagacaccatctgcggggtggggaacatgtcagcaaacgcctctgaccaagagaggacaccctggcatgtcactattaagcccaagagccaagagacctgccggggagccctcatctccgaccaatgggtcctgacagcggctcactgcttccgcgatggcaacgaccactccctatggagggtcaatgtgggagaccccaaatcccagtggggcaaagaattccttattgagaaggcagtgatttccccaggatttgatgtctttgccaaaaagaaccagggaatcctggagttctatggtgatgacatcgccctgctgaagctggcccagaaagtaaagatgtccacccatgccaggcccatctgccttccctgcaccatggaggccaatctggctctgcggagacctcaaggcagcacctgtagggaccatgagaatgaactgctgaacaaacagagtgttcctgctcattttgtcgccttgaatgggagcaaactgaacattaaccttaagatgggagtggagtggacaagctgtgccgaggtcgtctcccaagaaaaaaccatgttccccaacttgacagatgtcagggaggtggtgacagaccagtttctatgcagtgggacccaggaggatgagagtccctgcaagggtgtgaccaccactccattgtcttcggcccagcctcaaggatcctgctctctggagggggtagagatcaaaggtggctccttccgacttctccaagagggccaggcactggaatacgtgtgtccttctggcttctacccgtaccctgtgcagacacgtacctgcagatccacggggtcctggagcaccctgcagactcaagatcgaaaaactgtcaagaaggcagagtgcagagcaatccgctgtccacgaccacaggacttcgagaacggggaataccggccccggtctccctactacaatgtgagtgatgagatctctttccactgctatgacggttacactctccggggctctgccaatcgcacctgccaagtgaatggccggtggagtgggcagacagcgatctgtgacaacggagcggggtactgctccaacccaggcatccccattggcacaaggaaggtgggcagccggtaccgccttgaagacagcgtcacctaccactgcagccgggggcttaccctgcgtggctcccagcggcgaacatgtcaggaaggtggctcttggagcgggacggagccttcctgccaagactccttcatgtacgacacccctcaagaggtggccgaagctttcctgtcttccctgacggagaccatagaaggagtcgatgccgaggatgggcacagcccaggggaacaacagaagcggaggatcatcctagacccttcaggctccatgaacatctacctggtgctagatggatcagacagcattggggccggcaacttcacaggagccaaaaagtgtctagtcaacttaattgagaaggtggcaagttatggtgtgaagccaagatatgctctagtgacatatgccacataccccagaatttgggtcaaagtgtctgaccaagagagcagcaatgcagactgggtcacgaagaagctcagtgaaatcaattatgaagaccacaagttgaagtcagggactaacaccaagagggccctccaggcagtgtacagcatgatgagttggccagaggacatccctcctgaaggctggaaccgcacccgccatgtcatcatcctcatgaccgatggattgcacaacatgggcggggacccaattactgtcattgatgagatccgggacttgttatacatcggcaaggatcgtaaaaacccgagggaggattatctggatgtctatgtgtttggggttggacctttggtggaccaagtgaacatcaatgctttggcttccaagaaagacaatgagcaacatgtgttcaaagtcaaggatatggaaaacctggaagacgttttcttccaaatgattgatgaaagccagtctctgagtctctgtggcatggtttgggaacacagcaagggtaccgattaccacaagcaaccatggcaggccaagatctcagtcactcgcccttcgaagggacatgagagctgtatgggggctgtggtgtctgagtactttgtgctgacagcagcacattgttttactgtggacgacaaggaacactcaatcaaggtcagcgtgggagggaagaagcgggacctggagatagaaaaagtcctatttcaccccgactacaacattagcgagaaaaaagaagcaggaattcctgaattttatgactatgacgttgccctgatcaagctcaagaataagttgaattatgacccgactatcaggcccatttgtctcccctgcaccgagggaacaactcgagctttgaggcttcctccaactaccacttgccagcaacagaaggaagagctgctccctgcacaggatatcaaagctctgtttgtgtctgaggaggagaagaagctgactcggaaggaggtctacatcaagaatggggataagaaaggcagctgtgagagagatgctcaatatgccccaggctatgacaaagtcaaggacatctcggaggtggtcacccctcggttcctttgtactggaggagtgagtccctatgctgaccccaatacttgcagaggtgattctggcggccccttgatagttcacaagagaagtcgtttcattcaagttggtgtcatcagctggggagtagtggatgtctgcaaaaaccagaagcggcaaaagcaggtacctgctcacgcccgagactttcacgtcaacctcttccaagtgctgccctggctgaaggagaaactccaagatgaggatttgggttttctctaaggggtttcctgctggacaggggcgcgggattgaattaaaacagctgcgacaacactt

SEQ ID NO: 5 - DNA, 2767 bp, Mus musculus
gctccatcacacagtccatggaaagactgatcttttaaattgggggtagtggaggtggtggtctgtgcttgttaggaggggtctgggggctaagagggagctttgaaagggaagttctggcccttggtcagtcaagggtggggctcacatagtttctgtttcctcagttggcagttcagctggggccctccttcatgaatgttccgggaagcagtggctgcgtgcgcagggtaggctggccaggctgcagatgccagagcagattgcataaaaggttaggggacagtgggaaaggggtgtagccagatccagcatttgggtttcagtttggacaggaggtcaaataggcacccagagtgacctggagagggctttgggccactggactctctggtgctttccatgacaatggagagcccccagctctgcctcgtcctcttggtcttaggcttctcctctggaggtgtgagcgcaactccagtgcttgaggcccggccccaagtctcctgctctctggagggagtagagatcaaaggcggctcctttcaacttctccaaggcggtcaggccctggagtacctatgtccctctggcttctacccataccccgtgcagactcgaacctgcagatccacaggctcctggagcgacctgcagacccgagaccaaaagattgtccagaaggcggaatgcagagcaatacgctgcccacgaccgcaggactttgaaaatggggaattctggccccggtcccccttctacaacctgagtgaccagatttcttttcaatgctatgatggttacgttctccggggctctgctaatcgcacctgccaagagaatggccggtgggatgggcaaacagcaatttgtgatgatggagctggatactgtcccaatcccggtattcctattgggacaaggaaggtgggtagccaataccgccttgaagacattgttacttaccactgcagccggggacttgtcctgcgtggctcccagaagcgaaagtgtcaagaaggtggctcatggagtgggacagagccttcctgccaagattccttcatgtatgacagccctcaagaagtggccgaagcattcctatcctccctgacagagaccatcgaaggagccgatgctgaggatgggcacagcccaggagaacagcagaagaggaagattgtcctagacccctcgggctccatgaatatctacctggtgctagatggatcagacagcatcggaagcagcaacttcacaggggctaagcggtgcctcaccaacttgattgagaaggtggcgagttacggggtgaggccacgatatggtctcctgacatatgctacagtccccaaagtgttggtcagagtgtctgatgagaggagtagcgatgccgactgggtcacagagaagctcaaccaaatcagttatgaagaccacaagctgaagtcagggaccaacaccaagagggctctccaggctgtgtatagcatgatgagctgggcaggggatgccccgcctgaaggctggaatagaacccgccatgtcatcatcattatgactgatggcttgcacaacatgggtggaaaccctgtcactgtcattcaggacatccgagccttgctggacatcggcagggatcccaaaaatcccagggaggattacctggatgtgtatgtgtttggggtcgggcctctggtggactccgtgaacatcaatgccttagcttccaaaaaggacaatgagcatcatgtgtttaaagtcaaggatatggaagacctggagaatgttttctaccaaatgattgatgaaaccaaatctctgagtctctgtggcatggtgtgggagcataaaaaaggcaacgattatcataagcaaccatggcaagccaagatctcagtcactcgccctctgaaaggacatgagacctgtatgggggccgtggtgtctgagtacttcgtgctgacagcagcgcactgcttcatggtggatgatcagaaacattccatcaaggtcagcgtggggggtcagaggcgggacctggagattgaagaggtcctgttccaccccaaatacaatattaatgggaaaaaggcagaagggatccctgagttctatgattatgatgtggccctagtcaagctcaagaacaagctcaagtatggccagactctcaggcccatctgtctcccctgcacggagggaaccacacgagccttgaggcttcctcagacagccacctgcaagcagcacaaggaacagttgctccctgtgaaggatgtcaaagctctgtttgtatctgagcaagggaagagcctgactcggaaggaggtgtacatcaagaatggggacaagaaagccagttgtgagagagatgctacaaaggcccaaggctatgagaaggtcaaagatgcctctgaggtggtcactccacggttcctctgcacaggaggggtggatccctatgctgaccccaacacatgcaaaggagattccgggggccctctcattgttcacaagagaagccgcttcattcaagttggtgtgattagctggggagtagtagatgtctgcagagaccagaggcggcaacagctggtaccctcttatgcccgggacttccacatcaacctcttccaggtgctgccctggctaaaggacaagctcaaagatgaggatttgggttttctataaagagcttcctgcagggagagtgtgaggacagattaaagcagttacaataacaaaaaaaaaaaaaaaaaaaaaa

SEQ ID NO: 6 - DNA, 20 bp, Artificial sequence
  Synthetic Oligonucleotide
gctgagctgccagtcaagga

SEQ ID NO: 7 - DNA, 20 bp, Artificial sequence
  Synthetic Oligonucleotide
ggccccgctgagctgccagt

SEQ ID NO: 8 - DNA, 20 bp, Artificial sequence
  Synthetic Oligonucleotide
cggaacatccaagcgggagg

SEQ ID NO: 9 - DNA, 20 bp, Artificial sequence
  Synthetic Oligonucleotide
ctttcccggaacatccaagc

SEQ ID NO: 10 - DNA, 20 bp, Artificial sequence
  Synthetic Oligonucleotide
atctgtgttctggcacctgc

SEQ ID NO: 11 - DNA, 20 bp, Artificial sequence
  Synthetic Oligonucleotide
gtcacattcccttcccctgc

SEQ ID NO: 12 - DNA, 20 bp, Artificial sequence
  Synthetic Oligonucleotide
gacctggtcacattcccttc

SEQ ID NO: 13 - DNA, 20 bp, Artificial sequence
  Synthetic Oligonucleotide
gacctagacctggtcacatt

SEQ ID NO: 14 - DNA, 20 bp, Artificial sequence
  Synthetic Oligonucleotide
actccagacctagacctggt

SEQ ID NO: 15 - DNA, 20 bp, Artificial sequence
  Synthetic Oligonucleotide
gctgaaactccagacctaga

SEQ ID NO: 16 - DNA, 20 bp, Artificial sequence
  Synthetic Oligonucleotide
gtccaagctgaaactccaga

SEQ ID NO: 17 - DNA, 20 bp, Artificial sequence
  Synthetic Oligonucleotide
ctcagtgtccaagctgaaac

SEQ ID NO: 18 - DNA, 20 bp, Artificial sequence
  Synthetic Oligonucleotide
aggagagaagctgggcctgg

SEQ ID NO: 19 - DNA, 20 bp, Artificial sequence
  Synthetic Oligonucleotide
gaaggcaggagagaagctgg

SEQ ID NO: 20 - DNA, 20 bp, Artificial sequence
  Synthetic Oligonucleotide
gtggtggtcacacctccaga

SEQ ID NO: 21 - DNA, 20 bp, Artificial sequence
  Synthetic Oligonucleotide
ccctccagagagcaggatcc

SEQ ID NO: 22 - DNA, 20 bp, Artificial sequence
  Synthetic Oligonucleotide
tctaccccctccagagagca

SEQ ID NO: 23 - DNA, 20 bp, Artificial sequence
  Synthetic Oligonucleotide
ttgatctctaccccctccag

SEQ ID NO: 24 - DNA, 20 bp, Artificial sequence
  Synthetic Oligonucleotide
tggagaagtcggaaggagcc

SEQ ID NO: 25 - DNA, 20 bp, Artificial sequence
  Synthetic Oligonucleotide
ccctcttggagaagtcggaa

SEQ ID NO: 26 - DNA, 20 bp, Artificial sequence
  Synthetic Oligonucleotide
gcctggccctcttggagaag

SEQ ID NO: 27 - DNA, 20 bp, Artificial sequence
  Synthetic Oligonucleotide
tccagtgcctggccctcttg

SEQ ID NO: 28 - DNA, 20 bp, Artificial sequence
  Synthetic Oligonucleotide
agaagccagaaggacacacg

SEQ ID NO: 29 - DNA, 20 bp, Artificial sequence
  Synthetic Oligonucleotide
acgggtagaagccagaagga

SEQ ID NO: 30 - DNA, 20 bp, Artificial sequence
  Synthetic Oligonucleotide
cgtgtctgcacagggtacgg

SEQ ID NO: 31 - DNA, 20 bp, Artificial sequence
  Synthetic Oligonucleotide
agggtgctccaggaccccgt

SEQ ID NO: 32 - DNA, 20 bp, Artificial sequence
  Synthetic Oligonucleotide
ttgctctgcactctgccttc

SEQ ID NO: 33 - DNA, 20 bp, Artificial sequence
  Synthetic Oligonucleotide
tattccccgttctcgaagtc

SEQ ID NO: 34 - DNA, 20 bp, Artificial sequence
  Synthetic Oligonucleotide
cattgtagtagggagaccgg

SEQ ID NO: 35 - DNA, 20 bp, Artificial sequence
  Synthetic Oligonucleotide
cactcacattgtagtaggga

SEQ ID NO: 36 - DNA, 20 bp, Artificial sequence
  Synthetic Oligonucleotide
tctcatcactcacattgtag

SEQ ID NO: 37 - DNA, 20 bp, Artificial sequence
  Synthetic Oligonucleotide
aagagatctcatcactcaca

SEQ ID NO: 38 - DNA, 20 bp, Artificial sequence
  Synthetic Oligonucleotide
agtggaaagagatctcatca

SEQ ID NO: 39 - DNA, 20 bp, Artificial sequence
  Synthetic Oligonucleotide
catagcagtggaaagagatc

SEQ ID NO: 40 - DNA, 20 bp, Artificial sequence
  Synthetic Oligonucleotide
aaccgtcatagcagtggaaa

SEQ ID NO: 41 - DNA, 20 bp, Artificial sequence
  Synthetic Oligonucleotide
gagtgtaaccgtcatagcag

SEQ ID NO: 42 - DNA, 20 bp, Artificial sequence
  Synthetic Oligonucleotide
cccggagagtgtaaccgtca

SEQ ID NO: 43 - DNA, 20 bp, Artificial sequence
  Synthetic Oligonucleotide
cagagccccggagagtgtaa

SEQ ID NO: 44 - DNA, 20 bp, Artificial sequence
  Synthetic Oligonucleotide
gattggcagagccccggaga

SEQ ID NO: 45 - DNA, 20 bp, Artificial sequence
  Synthetic Oligonucleotide
aggtgcgattggcagagccc

SEQ ID NO: 46 - DNA, 20 bp, Artificial sequence
  Synthetic Oligonucleotide
cttggcaggtgcgattggca

SEQ ID NO: 47 - DNA, 20 bp, Artificial sequence
  Synthetic Oligonucleotide
cattcacttggcaggtgcga

SEQ ID NO: 48 - DNA, 20 bp, Artificial sequence
  Synthetic Oligonucleotide
atcgctgtctgcccactcca

SEQ ID NO: 49 - DNA, 20 bp, Artificial sequence
  Synthetic Oligonucleotide
tcacagatcgctgtctgccc

SEQ ID NO: 50 - DNA, 20 bp, Artificial sequence
  Synthetic Oligonucleotide
ccgttgtcacagatcgctgt

SEQ ID NO: 51 - DNA, 20 bp, Artificial sequence
  Synthetic Oligonucleotide
cccgctccgttgtcacagat

SEQ ID NO: 52 - DNA, 20 bp, Artificial sequence
  Synthetic Oligonucleotide
cagtaccccgctccgttgtc

SEQ ID NO: 53 - DNA, 20 bp, Artificial sequence
  Synthetic Oligonucleotide
ttggagcagtaccccgctcc

SEQ ID NO: 54 - DNA, 20 bp, Artificial sequence
  Synthetic Oligonucleotide
accttccttgtgccaatggg

SEQ ID NO: 55 - DNA, 20 bp, Artificial sequence
  Synthetic Oligonucleotide
ctgcccaccttccttgtgcc

SEQ ID NO: 56 - DNA, 20 bp, Artificial sequence
  Synthetic Oligonucleotide
cgctgtcttcaaggcggtac

SEQ ID NO: 57 - DNA, 20 bp, Artificial sequence
  Synthetic Oligonucleotide
gctgcagtggtaggtgacgc

SEQ ID NO: 58 - DNA, 20 bp, Artificial sequence
  Synthetic Oligonucleotide
cccccggctgcagtggtagg

SEQ ID NO: 59 - DNA, 20 bp, Artificial sequence
  Synthetic Oligonucleotide
ggtaagcccccggctgcagt

SEQ ID NO: 60 - DNA, 20 bp, Artificial sequence
  Synthetic Oligonucleotide
acgcagggtaagcccccggc

SEQ ID NO: 61 - DNA, 20 bp, Artificial sequence
  Synthetic Oligonucleotide
ggagccacgcagggtaagcc

SEQ ID NO: 62 - DNA, 20 bp, Artificial sequence
  Synthetic Oligonucleotide
gccgctgggagccacgcagg

SEQ ID NO: 63 - DNA, 20 bp, Artificial sequence
  Synthetic Oligonucleotide
caagagccaccttcctgaca

SEQ ID NO: 64 - DNA, 20 bp, Artificial sequence
  Synthetic Oligonucleotide
ccgctccaagagccaccttc

SEQ ID NO: 65 - DNA, 20 bp, Artificial sequence
  Synthetic Oligonucleotide
tccgtcccgctccaagagcc

SEQ ID NO: 66 - DNA, 20 bp, Artificial sequence
  Synthetic Oligonucleotide
gaaggctccgtcccgctcca

SEQ ID NO: 67 - DNA, 20 bp, Artificial sequence
  Synthetic Oligonucleotide
tggcaggaaggctccgtccc

SEQ ID NO: 68 - DNA, 20 bp, Artificial sequence
  Synthetic Oligonucleotide
gagtcttggcaggaaggctc

SEQ ID NO: 69 - DNA, 20 bp, Artificial sequence
  Synthetic Oligonucleotide
atgaaggagtcttggcagga

SEQ ID NO: 70 - DNA, 20 bp, Artificial sequence
  Synthetic Oligonucleotide
cttcggccacctcttgaggg

SEQ ID NO: 71 - DNA, 20 bp, Artificial sequence
  Synthetic Oligonucleotide
ggaaagcttcggccacctct

SEQ ID NO: 72 - DNA, 20 bp, Artificial sequence
  Synthetic Oligonucleotide
aagacaggaaagcttcggcc

SEQ ID NO: 73 - DNA, 20 bp, Artificial sequence
  Synthetic Oligonucleotide
tcagggaagacaggaaagct

SEQ ID NO: 74 - DNA, 20 bp, Artificial sequence
  Synthetic Oligonucleotide
tcgactccttctatggtctc

SEQ ID NO: 75 - DNA, 20 bp, Artificial sequence
  Synthetic Oligonucleotide
cttctgttgttcccctgggc

SEQ ID NO: 76 - DNA, 20 bp, Artificial sequence
  Synthetic Oligonucleotide
ttcatggagcctgaagggtc

SEQ ID NO: 77 - DNA, 20 bp, Artificial sequence
  Synthetic Oligonucleotide
tagatgttcatggagcctga

SEQ ID NO: 78 - DNA, 20 bp, Artificial sequence
  Synthetic Oligonucleotide
accaggtagatgttcatgga

SEQ ID NO: 79 - DNA, 20 bp, Artificial sequence
  Synthetic Oligonucleotide
tctagcaccaggtagatgtt

SEQ ID NO: 80 - DNA, 20 bp, Artificial sequence
  Synthetic Oligonucleotide
gatccatctagcaccaggta

SEQ ID NO: 81 - DNA, 20 bp, Artificial sequence
  Synthetic Oligonucleotide
ctgtctgatccatctagcac

SEQ ID NO: 82 - DNA, 20 bp, Artificial sequence
  Synthetic Oligonucleotide
ccaatgctgtctgatccatc

SEQ ID NO: 83 - DNA, 20 bp, Artificial sequence
  Synthetic Oligonucleotide
tttggctcctgtgaagttgc

SEQ ID NO: 84 - DNA, 20 bp, Artificial sequence
  Synthetic Oligonucleotide
acactttttggctcctgtga

SEQ ID NO: 85 - DNA, 20 bp, Artificial sequence
  Synthetic Oligonucleotide
gactagacactttttggctc

SEQ ID NO: 86 - DNA, 20 bp, Artificial sequence
  Synthetic Oligonucleotide
taagttgactagacactttt

SEQ ID NO: 87 - DNA, 20 bp, Artificial sequence
  Synthetic Oligonucleotide
ctcaattaagttgactagac

SEQ ID NO: 88 - DNA, 20 bp, Artificial sequence
  Synthetic Oligonucleotide
caccttctcaattaagttga

SEQ ID NO: 89 - DNA, 20 bp, Artificial sequence
  Synthetic Oligonucleotide
acttgccaccttctcaatta

SEQ ID NO: 90 - DNA, 20 bp, Artificial sequence
  Synthetic Oligonucleotide
accataacttgccaccttct

SEQ ID NO: 91 - DNA, 20 bp, Artificial sequence
  Synthetic Oligonucleotide
cttcacaccataacttgcca

SEQ ID NO: 92 - DNA, 20 bp, Artificial sequence
  Synthetic Oligonucleotide
tcttggcttcacaccataac

SEQ ID NO: 93 - DNA, 20 bp, Artificial sequence
  Synthetic Oligonucleotide
atgtggcatatgtcactaga

SEQ ID NO: 94 - DNA, 20 bp, Artificial sequence
  Synthetic Oligonucleotide
cagacactttgacccaaatt

SEQ ID NO: 95 - DNA, 20 bp, Artificial sequence
  Synthetic Oligonucleotide
ggtcttcataattgatttca

SEQ ID NO: 96 - DNA, 20 bp, Artificial sequence
  Synthetic Oligonucleotide
acttgtggtcttcataattg

SEQ ID NO: 97 - DNA, 20 bp, Artificial sequence
  Synthetic Oligonucleotide
acttcaacttgtggtcttca

SEQ ID NO: 98 - DNA, 20 bp, Artificial sequence
  Synthetic Oligonucleotide
tccctgacttcaacttgtgg

SEQ ID NO: 99 - DNA, 20 bp, Artificial sequence
  Synthetic Oligonucleotide
tgttagtccctgacttcaac

SEQ ID NO: 100 - DNA, 20 bp, Artificial sequence
  Synthetic Oligonucleotide
tcttggtgttagtccctgac

SEQ ID NO: 101 - DNA, 20 bp, Artificial sequence
  Synthetic Oligonucleotide
tgtacactgcctggagggcc

SEQ ID NO: 102 - DNA, 20 bp, Artificial sequence
  Synthetic Oligonucleotide
tcatgctgtacactgcctgg

SEQ ID NO: 103 - DNA, 20 bp, Artificial sequence
  Synthetic Oligonucleotide
gttccagccttcaggaggga

SEQ ID NO: 104 - DNA, 20 bp, Artificial sequence
  Synthetic Oligonucleotide
ggtgcggttccagccttcag

SEQ ID NO: 105 - DNA, 20 bp, Artificial sequence
  Synthetic Oligonucleotide
atggcgggtgcggttccagc

SEQ ID NO: 106 - DNA, 20 bp, Artificial sequence
  Synthetic Oligonucleotide
gatgacatggcgggtgcggt

SEQ ID NO: 107 - DNA, 20 bp, Artificial sequence
  Synthetic Oligonucleotide
gaggatgatgacatggcggg

SEQ ID NO: 108 - DNA, 20 bp, Artificial sequence
  Synthetic Oligonucleotide
cccatgttgtgcaatccatc

SEQ ID NO: 109 - DNA, 20 bp, Artificial sequence
  Synthetic Oligonucleotide
tccccgcccatgttgtgcaa

SEQ ID NO: 110 - DNA, 20 bp, Artificial sequence
  Synthetic Oligonucleotide
attgggtccccgcccatgtt

SEQ ID NO: 111 - DNA, 20 bp, Artificial sequence
  Synthetic Oligonucleotide
acagtaattgggtccccgcc

SEQ ID NO: 112 - DNA, 20 bp, Artificial sequence
  Synthetic Oligonucleotide
tcaatgacagtaattgggtc

SEQ ID NO: 113 - DNA, 20 bp, Artificial sequence
  Synthetic Oligonucleotide
atctcatcaatgacagtaat

SEQ ID NO: 114 - DNA, 20 bp, Artificial sequence
  Synthetic Oligonucleotide
tcccggatctcatcaatgac

SEQ ID NO: 115 - DNA, 20 bp, Artificial sequence
  Synthetic Oligonucleotide
acatccagataatcctccct

SEQ ID NO: 116 - DNA, 20 bp, Artificial sequence
  Synthetic Oligonucleotide
acatagacatccagataatc

SEQ ID NO: 117 - DNA, 20 bp, Artificial sequence
  Synthetic Oligonucleotide
ccaaacacatagacatccag

SEQ ID NO: 118 - DNA, 20 bp, Artificial sequence
  Synthetic Oligonucleotide
agcattgatgttcacttggt

SEQ ID NO: 119 - DNA, 20 bp, Artificial sequence
  Synthetic Oligonucleotide
agccaaagcattgatgttca

SEQ ID NO: 120 - DNA, 20 bp, Artificial sequence
  Synthetic Oligonucleotide
cttggaagccaaagcattga

SEQ ID NO: 121 - DNA, 20 bp, Artificial sequence
  Synthetic Oligonucleotide
gtctttcttggaagccaaag

SEQ ID NO: 122 - DNA, 20 bp, Artificial sequence
  Synthetic Oligonucleotide
ctcattgtctttcttggaag

SEQ ID NO: 123 - DNA, 20 bp, Artificial sequence
  Synthetic Oligonucleotide
atgttgctcattgtctttct

SEQ ID NO: 124 - DNA, 20 bp, Artificial sequence
  Synthetic Oligonucleotide
gaacacatgttgctcattgt

SEQ ID NO: 125 - DNA, 20 bp, Artificial sequence
  Synthetic Oligonucleotide
gactttgaacacatgttgct

SEQ ID NO: 126 - DNA, 20 bp, Artificial sequence
  Synthetic Oligonucleotide
atccttgactttgaacacat

SEQ ID NO: 127 - DNA, 20 bp, Artificial sequence
  Synthetic Oligonucleotide
ttccatatccttgactttga

SEQ ID NO: 128 - DNA, 20 bp, Artificial sequence
  Synthetic Oligonucleotide
caggttttccatatccttga

SEQ ID NO: 129 - DNA, 20 bp, Artificial sequence
  Synthetic Oligonucleotide
ctcagagactggctttcatc

SEQ ID NO: 130 - DNA, 20 bp, Artificial sequence
  Synthetic Oligonucleotide
cagagactcagagactggct

SEQ ID NO: 131 - DNA, 20 bp, Artificial sequence
  Synthetic Oligonucleotide
atgccacagagactcagaga

SEQ ID NO: 132 - DNA, 20 bp, Artificial sequence
  Synthetic Oligonucleotide
caaaccatgccacagagact

SEQ ID NO: 133 - DNA, 20 bp, Artificial sequence
  Synthetic Oligonucleotide
tgttcccaaaccatgccaca

SEQ ID NO: 134 - DNA, 20 bp, Artificial sequence
  Synthetic Oligonucleotide
ttgtggtaatcggtaccctt

SEQ ID NO: 135 - DNA, 20 bp, Artificial sequence
  Synthetic Oligonucleotide
ggttgcttgtggtaatcggt

SEQ ID NO: 136 - DNA, 20 bp, Artificial sequence
  Synthetic Oligonucleotide
tgccatggttgcttgtggta

SEQ ID NO: 137 - DNA, 20 bp, Artificial sequence
  Synthetic Oligonucleotide
ttggcctgccatggttgctt

SEQ ID NO: 138 - DNA, 20 bp, Artificial sequence
  Synthetic Oligonucleotide
gagatcttggcctgccatgg

SEQ ID NO: 139 - DNA, 20 bp, Artificial sequence
  Synthetic Oligonucleotide
acagcccccatacagctctc

SEQ ID NO: 140 - DNA, 20 bp, Artificial sequence
  Synthetic Oligonucleotide
gacaccacagcccccataca

SEQ ID NO: 141 - DNA, 20 bp, Artificial sequence
  Synthetic Oligonucleotide
tactcagacaccacagcccc

SEQ ID NO: 142 - DNA, 20 bp, Artificial sequence
  Synthetic Oligonucleotide
acaaagtactcagacaccac

SEQ ID NO: 143 - DNA, 20 bp, Artificial sequence
  Synthetic Oligonucleotide
gtcagcacaaagtactcaga

SEQ ID NO: 144 - DNA, 20 bp, Artificial sequence
  Synthetic Oligonucleotide
ttgattgagtgttccttgtc

SEQ ID NO: 145 - DNA, 20 bp, Artificial sequence
  Synthetic Oligonucleotide
ctgaccttgattgagtgttc

SEQ ID NO: 146 - DNA, 20 bp, Artificial sequence
  Synthetic Oligonucleotide
tatctccaggtcccgcttct

SEQ ID NO: 147 - DNA, 20 bp, Artificial sequence
  Synthetic Oligonucleotide
gaattcctgcttcttttttc

SEQ ID NO: 148 - DNA, 20 bp, Artificial sequence
  Synthetic Oligonucleotide
attcaggaattcctgcttct

SEQ ID NO: 149 - DNA, 20 bp, Artificial sequence
  Synthetic Oligonucleotide
cataaaattcaggaattcct

SEQ ID NO: 150 - DNA, 20 bp, Artificial sequence
  Synthetic Oligonucleotide
catagtcataaaattcagga

SEQ ID NO: 151 - DNA, 20 bp, Artificial sequence
  Synthetic Oligonucleotide
tgagcttgatcagggcaacg

SEQ ID NO: 152 - DNA, 20 bp, Artificial sequence
  Synthetic Oligonucleotide
tattcttgagcttgatcagg

SEQ ID NO: 153 - DNA, 20 bp, Artificial sequence
  Synthetic Oligonucleotide
gacaaatgggcctgatagtc

SEQ ID NO: 154 - DNA, 20 bp, Artificial sequence
  Synthetic Oligonucleotide
gttgttccctcggtgcaggg

SEQ ID NO: 155 - DNA, 20 bp, Artificial sequence
  Synthetic Oligonucleotide
gctcgagttgttccctcggt

SEQ ID NO: 156 - DNA, 20 bp, Artificial sequence
  Synthetic Oligonucleotide
ctcaaagctcgagttgttcc

SEQ ID NO: 157 - DNA, 20 bp, Artificial sequence
  Synthetic Oligonucleotide
ggaagcctcaaagctcgagt

SEQ ID NO: 158 - DNA, 20 bp, Artificial sequence
  Synthetic Oligonucleotide
gttggaggaagcctcaaagc

SEQ ID NO: 159 - DNA, 20 bp, Artificial sequence
  Synthetic Oligonucleotide
gtggtagttggaggaagcct

SEQ ID NO: 160 - DNA, 20 bp, Artificial sequence
  Synthetic Oligonucleotide
tggcaagtggtagttggagg

SEQ ID NO: 161 - DNA, 20 bp, Artificial sequence
  Synthetic Oligonucleotide
tgttgctggcaagtggtagt

SEQ ID NO: 162 - DNA, 20 bp, Artificial sequence
  Synthetic Oligonucleotide
tccagctcactcccctgttg

SEQ ID NO: 163 - DNA, 20 bp, Artificial sequence
  Synthetic Oligonucleotide
taaggatccagctcactccc

SEQ ID NO: 164 - DNA, 20 bp, Artificial sequence
  Synthetic Oligonucleotide
cagaaataaggatccagctc

SEQ ID NO: 165 - DNA, 20 bp, Artificial sequence
  Synthetic Oligonucleotide
agggaccagaaataaggatc

SEQ ID NO: 166 - DNA, 20 bp, Artificial sequence
  Synthetic Oligonucleotide
ccacttagggaccagaaata

SEQ ID NO: 167 - DNA, 20 bp, Artificial sequence
  Synthetic Oligonucleotide
tccaggactctccccttcag

SEQ ID NO: 168 - DNA, 20 bp, Artificial sequence
  Synthetic Oligonucleotide
aagtcccaccctttgctgcc

SEQ ID NO: 169 - DNA, 20 bp, Artificial sequence
  Synthetic Oligonucleotide
ctgcagaagtcccacccttt

SEQ ID NO: 170 - DNA, 20 bp, Artificial sequence
  Synthetic Oligonucleotide
cagaaactgcagaagtccca

SEQ ID NO: 171 - DNA, 20 bp, Artificial sequence
  Synthetic Oligonucleotide
aacctctgcactctgccttc

SEQ ID NO: 172 - DNA, 20 bp, Artificial sequence
  Synthetic Oligonucleotide
ccctcaaacctctgcactct

SEQ ID NO: 173 - DNA, 20 bp, Artificial sequence
  Synthetic Oligonucleotide
tcattgccctcaaacctctg

SEQ ID NO: 174 - DNA, 20 bp, Artificial sequence
  Synthetic Oligonucleotide
ccacactcattgccctcaaa

SEQ ID NO: 175 - DNA, 20 bp, Artificial sequence
  Synthetic Oligonucleotide
cactgcccacactcattgcc

SEQ ID NO: 176 - DNA, 20 bp, Artificial sequence
  Synthetic Oligonucleotide
ttaggccactgcccacactc

SEQ ID NO: 177 - DNA, 20 bp, Artificial sequence
  Synthetic Oligonucleotide
ctagtcctgaccttgctgcc

SEQ ID NO: 178 - DNA, 20 bp, Artificial sequence
  Synthetic Oligonucleotide
ctcatcctagtcctgacctt

SEQ ID NO: 179 - DNA, 20 bp, Artificial sequence
  Synthetic Oligonucleotide
cctagtctcatcctagtcct

SEQ ID NO: 180 - DNA, 20 bp, Artificial sequence
  Synthetic Oligonucleotide
accctgcctagtctcatcct

SEQ ID NO: 181 - DNA, 20 bp, Artificial sequence
  Synthetic Oligonucleotide
cttgtcaccctgcctagtct

SEQ ID NO: 182 - DNA, 20 bp, Artificial sequence
  Synthetic Oligonucleotide
gcccaccttgtcaccctgcc

SEQ ID NO: 183 - DNA, 20 bp, Artificial sequence
  Synthetic Oligonucleotide
cctaaaactgctcctactcc

SEQ ID NO: 184 - DNA, 20 bp, Artificial sequence
  Synthetic Oligonucleotide
gagtcagaaatgaggtcaaa

SEQ ID NO: 185 - DNA, 20 bp, Artificial sequence
  Synthetic Oligonucleotide
ccctactcccatttcacctt

SEQ ID NO: 186 - DNA, 20 bp, Artificial sequence
  Synthetic Oligonucleotide
tgttgtgcaatcctgcagaa

SEQ ID NO: 187 - DNA, 20 bp, Artificial sequence
  Synthetic Oligonucleotide
aaaggctgatgaagcctggc

SEQ ID NO: 188 - DNA, 20 bp, Artificial sequence
  Synthetic Oligonucleotide
cctttgaccacaaagtggcc

SEQ ID NO: 189 - DNA, 20 bp, Artificial sequence
  Synthetic Oligonucleotide
aggtaccacctctttgtggg

SEQ ID NO: 190 - DNA, 20 bp, Artificial sequence
  Synthetic Oligonucleotide
tggtggtcacacctgaagag

SEQ ID NO: 191 - DNA, 20 bp, Artificial sequence
  Synthetic Oligonucleotide
gcagggagcagctcttcctt

SEQ ID NO: 192 - DNA, 20 bp, Artificial sequence
  Synthetic Oligonucleotide
tcctgtgcagggagcagctc

SEQ ID NO: 193 - DNA, 20 bp, Artificial sequence
  Synthetic Oligonucleotide
ttgatatcctgtgcagggag

SEQ ID NO: 194 - DNA, 20 bp, Artificial sequence
  Synthetic Oligonucleotide
agagctttgatatcctgtgc

SEQ ID NO: 195 - DNA, 20 bp, Artificial sequence
  Synthetic Oligonucleotide
acaaacagagctttgatatc

SEQ ID NO: 196 - DNA, 20 bp, Artificial sequence
  Synthetic Oligonucleotide
tcagacacaaacagagcttt

SEQ ID NO: 197 - DNA, 20 bp, Artificial sequence
  Synthetic Oligonucleotide
tcctcctcagacacaaacag

SEQ ID NO: 198 - DNA, 20 bp, Artificial sequence
  Synthetic Oligonucleotide
acctccttccgagtcagctt

SEQ ID NO: 199 - DNA, 20 bp, Artificial sequence
  Synthetic Oligonucleotide
atgtagacctccttccgagt

SEQ ID NO: 200 - DNA, 20 bp, Artificial sequence
  Synthetic Oligonucleotide
ttcttgatgtagacctcctt

SEQ ID NO: 201 - DNA, 20 bp, Artificial sequence
  Synthetic Oligonucleotide
tccccattcttgatgtagac

SEQ ID NO: 202 - DNA, 20 bp, Artificial sequence
  Synthetic Oligonucleotide
ttcttatccccattcttgat

SEQ ID NO: 203 - DNA, 20 bp, Artificial sequence
  Synthetic Oligonucleotide
ctgcctttcttatccccatt

SEQ ID NO: 204 - DNA, 20 bp, Artificial sequence
  Synthetic Oligonucleotide
tcacagctgcctttcttatc

SEQ ID NO: 205 - DNA, 20 bp, Artificial sequence
  Synthetic Oligonucleotide
tctctctcacagctgccttt

SEQ ID NO: 206 - DNA, 20 bp, Artificial sequence
  Synthetic Oligonucleotide
tgagcatctctctcacagct

SEQ ID NO: 207 - DNA, 20 bp, Artificial sequence
  Synthetic Oligonucleotide
gcatattgagcatctctctc

SEQ ID NO: 208 - DNA, 20 bp, Artificial sequence
  Synthetic Oligonucleotide
tgactttgtcatagcctggg

SEQ ID NO: 209 - DNA, 20 bp, Artificial sequence
  Synthetic Oligonucleotide
tgtccttgactttgtcatag

SEQ ID NO: 210 - DNA, 20 bp, Artificial sequence
  Synthetic Oligonucleotide
cagtacaaaggaaccgaggg

SEQ ID NO: 211 - DNA, 20 bp, Artificial sequence
  Synthetic Oligonucleotide
ctcctccagtacaaaggaac

SEQ ID NO: 212 - DNA, 20 bp, Artificial sequence
  Synthetic Oligonucleotide
gactcactcctccagtacaa

SEQ ID NO: 213 - DNA, 20 bp, Artificial sequence
  Synthetic Oligonucleotide
catagggactcactcctcca

SEQ ID NO: 214 - DNA, 20 bp, Artificial sequence
  Synthetic Oligonucleotide
ggtcagcatagggactcact

SEQ ID NO: 215 - DNA, 20 bp, Artificial sequence
  Synthetic Oligonucleotide
tcacctctgcaagtattggg

SEQ ID NO: 216 - DNA, 20 bp, Artificial sequence
  Synthetic Oligonucleotide
ccagaatcacctctgcaagt

SEQ ID NO: 217 - DNA, 20 bp, Artificial sequence
  Synthetic Oligonucleotide
gggccgccagaatcacctct

SEQ ID NO: 218 - DNA, 20 bp, Artificial sequence
  Synthetic Oligonucleotide
ctcttgtgaactatcaaggg

SEQ ID NO: 219 - DNA, 20 bp, Artificial sequence
  Synthetic Oligonucleotide
cgacttctcttgtgaactat

SEQ ID NO: 220 - DNA, 20 bp, Artificial sequence
  Synthetic Oligonucleotide
atgaaacgacttctcttgtg

SEQ ID NO: 221 - DNA, 20 bp, Artificial sequence
  Synthetic Oligonucleotide
acttgaatgaaacgacttct

SEQ ID NO: 222 - DNA, 20 bp, Artificial sequence
  Synthetic Oligonucleotide
acaccaacttgaatgaaacg

SEQ ID NO: 223 - DNA, 20 bp, Artificial sequence
  Synthetic Oligonucleotide
tccactactccccagctgat

SEQ ID NO: 224 - DNA, 20 bp, Artificial sequence
  Synthetic Oligonucleotide
cagacatccactactcccca

SEQ ID NO: 225 - DNA, 20 bp, Artificial sequence
  Synthetic Oligonucleotide
tttttgcagacatccactac

SEQ ID NO: 226 - DNA, 20 bp, Artificial sequence
  Synthetic Oligonucleotide
ttctggtttttgcagacatc

SEQ ID NO: 227 - DNA, 20 bp, Artificial sequence
  Synthetic Oligonucleotide
tgccgcttctggtttttgca

SEQ ID NO: 228 - DNA, 20 bp, Artificial sequence
  Synthetic Oligonucleotide
tgcttttgccgcttctggtt

SEQ ID NO: 229 - DNA, 20 bp, Artificial sequence
  Synthetic Oligonucleotide
ggtacctgcttttgccgctt

SEQ ID NO: 230 - DNA, 20 bp, Artificial sequence
  Synthetic Oligonucleotide
tgagcaggtacctgcttttg

SEQ ID NO: 231 - DNA, 20 bp, Artificial sequence
  Synthetic Oligonucleotide
ttcagccagggcagcacttg

SEQ ID NO: 232 - DNA, 20 bp, Artificial sequence
  Synthetic Oligonucleotide
ttctccttcagccagggcag

SEQ ID NO: 233 - DNA, 20 bp, Artificial sequence
  Synthetic Oligonucleotide
tggagtttctccttcagcca

SEQ ID NO: 234 - DNA, 20 bp, Artificial sequence
  Synthetic Oligonucleotide
tcatcttggagtttctcctt

SEQ ID NO: 235 - DNA, 20 bp, Artificial sequence
  Synthetic Oligonucleotide
aaatcctcatcttggagttt

SEQ ID NO: 236 - DNA, 20 bp, Artificial sequence
  Synthetic Oligonucleotide
aaacccaaatcctcatcttg

SEQ ID NO: 237 - DNA, 20 bp, Artificial sequence
  Synthetic Oligonucleotide
gtccagcaggaaacccctta

SEQ ID NO: 238 - DNA, 20 bp, Artificial sequence
  Synthetic Oligonucleotide
gcccctgtccagcaggaaac

SEQ ID NO: 239 - DNA, 20 bp, Artificial sequence
  Synthetic Oligonucleotide
agctgttttaattcaatccc

SEQ ID NO: 240 - DNA, 20 bp, Artificial sequence
  Synthetic Oligonucleotide
aacttgccacctgtgggtga

SEQ ID NO: 241 - DNA, 20 bp, Artificial sequence
  Synthetic Oligonucleotide
tcaccttatccccattcttg

SEQ ID NO: 242 - DNA, 20 bp, Artificial sequence
  Synthetic Oligonucleotide
tcaactttcacaaaccacca

SEQ ID NO: 243 - DNA, 20 bp, Artificial sequence
  Synthetic Oligonucleotide
ccgccagaatcacctgcaag

SEQ ID NO: 244 - DNA, 20 bp, Artificial sequence
  Synthetic Oligonucleotide
aggaggaatgaagaaggctt

SEQ ID NO: 245 - DNA, 20 bp, Artificial sequence
  Synthetic Oligonucleotide
gcctttcctcagggatctgg

SEQ ID NO: 246 - DNA, 20 bp, Artificial sequence
  Synthetic Oligonucleotide
aaatgtctgggagtgtcagg

SEQ ID NO: 247 - DNA, 20 bp, Artificial sequence
  Synthetic Oligonucleotide
gcctagagtgcctccttagg

SEQ ID NO: 248 - DNA, 20 bp, Artificial sequence
  Synthetic Oligonucleotide
ggcatctccccagataggaa

SEQ ID NO: 249 - DNA, 20 bp, Artificial sequence
  Synthetic Oligonucleotide
agggagctagtcctggaaga

SEQ ID NO: 250 - DNA, 20 bp, Artificial sequence
  Synthetic Oligonucleotide
acacctgaagagaaaggctg

SEQ ID NO: 251 - DNA, 20 bp, Artificial sequence
  Synthetic Oligonucleotide
ccctttgaccacaaagtggc

SEQ ID NO: 252 - DNA, 20 bp, Artificial sequence
  Synthetic Oligonucleotide
gccctcaaggtagtctcatg

SEQ ID NO: 253 - DNA, 20 bp, Artificial sequence
  Synthetic Oligonucleotide
aagggaaggaggacagaata

SEQ ID NO: 254 - DNA, 20 bp, Artificial sequence
  Synthetic Oligonucleotide
aaaggccaaggagggatgct

SEQ ID NO: 255 - DNA, 20 bp, Artificial sequence
  Synthetic Oligonucleotide
agaggtcccttctgaccatc

SEQ ID NO: 256 - DNA, 20 bp, Artificial sequence
  Synthetic Oligonucleotide
gctgggacaggagagaggtc

SEQ ID NO: 257 - DNA, 20 bp, Artificial sequence
  Synthetic Oligonucleotide
tcaaatgtctgggagtgtca

SEQ ID NO: 258 - DNA, 20 bp, Artificial sequence
  Synthetic Oligonucleotide
agaaggagaatgtgctgaaa

SEQ ID NO: 259 - DNA, 20 bp, Artificial sequence
  Synthetic Oligonucleotide
tgctgaccacttggcatctc

SEQ ID NO: 260 - DNA, 20 bp, Artificial sequence
  Synthetic Oligonucleotide
caactttcacaaaccaccat

SEQ ID NO: 261 - DNA, 20 bp, Artificial sequence
  Synthetic Oligonucleotide
agctctgtgattctaaggtt

SEQ ID NO: 262 - DNA, 20 bp, Artificial sequence
  Synthetic Oligonucleotide
ccacctgtgggtgaggagaa

SEQ ID NO: 263 - DNA, 20 bp, Artificial sequence
  Synthetic Oligonucleotide
gaggactcacttgaatgaaa

SEQ ID NO: 264 - DNA, 20 bp, Artificial sequence
  Synthetic Oligonucleotide
tggaatgatcagggagctag

SEQ ID NO: 265 - DNA, 20 bp, Artificial sequence
  Synthetic Oligonucleotide
gtcccttctccattttcccc

SEQ ID NO: 266 - DNA, 20 bp, Artificial sequence
  Synthetic Oligonucleotide
tcaactttttaagttaatca

SEQ ID NO: 267 - DNA, 20 bp, Artificial sequence
  Synthetic Oligonucleotide
gggtgaggagaacaaggcgc

SEQ ID NO: 268 - DNA, 20 bp, Artificial sequence
  Synthetic Oligonucleotide
cttccaagccatcttttaac

SEQ ID NO: 269 - DNA, 20 bp, Artificial sequence
  Synthetic Oligonucleotide
aggactcacttgaatgaaac

SEQ ID NO: 270 - DNA, 20 bp, Artificial sequence
  Synthetic Oligonucleotide
ttccaggcaactagagcttc

SEQ ID NO: 271 - DNA, 20 bp, Artificial sequence
  Synthetic Oligonucleotide
cagagtccagccactgtttg

SEQ ID NO: 272 - DNA, 20 bp, Artificial sequence
  Synthetic Oligonucleotide
ccaacctgcagaggcagtgg

SEQ ID NO: 273 - DNA, 20 bp, Artificial sequence
  Synthetic Oligonucleotide
tgcaaggagaggagaagctg

SEQ ID NO: 274 - DNA, 20 bp, Artificial sequence
  Synthetic Oligonucleotide
ctaggcaggttactcaccca

SEQ ID NO: 275 - DNA, 20 bp, Artificial sequence
  Synthetic Oligonucleotide
caccataacttgccacctgt

SEQ ID NO: 276 - DNA, 20 bp, Artificial sequence
  Synthetic Oligonucleotide
taggtaccacctctttgtgg

SEQ ID NO: 277 - DNA, 20 bp, Artificial sequence
  Synthetic Oligonucleotide
cttgacctcacctcccccaa

SEQ ID NO: 278 - DNA, 20 bp, Artificial sequence
  Synthetic Oligonucleotide
ccacctctttgtgggcagct

SEQ ID NO: 279 - DNA, 20 bp, Artificial sequence
  Synthetic Oligonucleotide
ttcacaaaccaccatctctt

SEQ ID NO: 280 - DNA, 20 bp, Artificial sequence
  Synthetic Oligonucleotide
ttctcacctccgttgtcaca

SEQ ID NO: 281 - DNA, 20 bp, Artificial sequence
  Synthetic Oligonucleotide
gaaagtgggaggtgttgcct

SEQ ID NO: 282 - DNA, 20 bp, Artificial sequence
  Synthetic Oligonucleotide
acagcaggaagggaaggtta

SEQ ID NO: 283 - DNA, 20 bp, Artificial sequence
  Synthetic Oligonucleotide
catgctgaccacttggcatc

SEQ ID NO: 284 - DNA, 20 bp, Artificial sequence
  Synthetic Oligonucleotide
ggtcaccttggcaggaaggc

SEQ ID NO: 285 - DNA, 20 bp, Artificial sequence
  Synthetic Oligonucleotide
gtatagtgttacaagtggac

SEQ ID NO: 286 - DNA, 20 bp, Artificial sequence
  Synthetic Oligonucleotide
ggacttccctttgaccacaa

SEQ ID NO: 287 - DNA, 20 bp, Artificial sequence
  Synthetic Oligonucleotide
tcaccttgacctcacctccc

SEQ ID NO: 288 - DNA, 20 bp, Artificial sequence
  Synthetic Oligonucleotide
tagagtgcctccttaggatg

SEQ ID NO: 289 - DNA, 20 bp, Artificial sequence
  Synthetic Oligonucleotide
tgacttcaacttgtggtctg

SEQ ID NO: 290 - DNA, 20 bp, Artificial sequence
  Synthetic Oligonucleotide
cagagaaggagaatgtgctg

SEQ ID NO: 291 - DNA, 20 bp, Artificial sequence
  Synthetic Oligonucleotide
agggagcagctcttcctctg

SEQ ID NO: 292 - DNA, 20 bp, Artificial sequence
  Synthetic Oligonucleotide
tgttcccctgggtgccagga

SEQ ID NO: 293 - DNA, 20 bp, Artificial sequence
  Synthetic Oligonucleotide
ggcctggctgttttcaagcc

SEQ ID NO: 294 - DNA, 20 bp, Artificial sequence
  Synthetic Oligonucleotide
gactggctttcatctggcag

SEQ ID NO: 295 - DNA, 20 bp, Artificial sequence
  Synthetic Oligonucleotide
gaaggctttccaggcaacta

SEQ ID NO: 296 - DNA, 20 bp, Artificial sequence
  Synthetic Oligonucleotide
tcacttgaatgaaacgactt

SEQ ID NO: 297 - DNA, 20 bp, Artificial sequence
  Synthetic Oligonucleotide
ggccccaaaaggccaaggag

SEQ ID NO: 298 - DNA, 20 bp, Artificial sequence
  Synthetic Oligonucleotide
aatcacctgcaaggagagga

SEQ ID NO: 299 - DNA, 20 bp, Artificial sequence
  Synthetic Oligonucleotide
gaccttcagttgcatcctta

SEQ ID NO: 300 - DNA, 20 bp, Artificial sequence
  Synthetic Oligonucleotide
tgatgaagcctggccccaaa

SEQ ID NO: 301 - DNA, 20 bp, Artificial sequence
  Synthetic Oligonucleotide
tagaaagtgggaggtgttgc

SEQ ID NO: 302 - DNA, 20 bp, Artificial sequence
  Synthetic Oligonucleotide
cccatccctgactggtctgg

SEQ ID NO: 303 - DNA, 20 bp, Artificial sequence
  Synthetic Oligonucleotide
ccatgggtatagtgttacaa

SEQ ID NO: 304 - DNA, 20 bp, Artificial sequence
  Synthetic Oligonucleotide
gtgttctcttgacttccagg

SEQ ID NO: 305 - DNA, 20 bp, Artificial sequence
  Synthetic Oligonucleotide
ggcctgctcctcaccccagt

SEQ ID NO: 306 - DNA, 20 bp, Artificial sequence
  Synthetic Oligonucleotide
gaggcctggctgttttcaag

SEQ ID NO: 307 - DNA, 20 bp, Artificial sequence
  Synthetic Oligonucleotide
gactctccccttcagtacct

SEQ ID NO: 308 - DNA, 20 bp, Artificial sequence
  Synthetic Oligonucleotide
catgggtatagtgttacaag

SEQ ID NO: 309 - DNA, 20 bp, Artificial sequence
  Synthetic Oligonucleotide
gaaggagaatgtgctgaaaa

SEQ ID NO: 310 - DNA, 20 bp, Artificial sequence
  Synthetic Oligonucleotide
tcacctggtcttccaagcca

SEQ ID NO: 311 - DNA, 20 bp, Artificial sequence
  Synthetic Oligonucleotide
ctccccagataggaaaggga

SEQ ID NO: 312 - DNA, 20 bp, Artificial sequence
  Synthetic Oligonucleotide
ggactcacttgaatgaaacg

SEQ ID NO: 313 - DNA, 20 bp, Artificial sequence
  Synthetic Oligonucleotide
ggccgccagaatcacctgca

SEQ ID NO: 314 - DNA, 20 bp, Artificial sequence
  Synthetic Oligonucleotide
ctcacttgaatgaaacgact

SEQ ID NO: 315 - DNA, 20 bp, Artificial sequence
  Synthetic Oligonucleotide
ctttcccagcctttcctcag

SEQ ID NO: 316 - DNA, 20 bp, Artificial sequence
  Synthetic Oligonucleotide
agaaagtgggaggtgttgcc

SEQ ID NO: 317 - DNA, 20 bp, Artificial sequence
  Synthetic Oligonucleotide
gtcgcagctgttttaattca

SEQ ID NO: 318 - DNA, 20 bp, Artificial sequence
  Synthetic Oligonucleotide
ccaggactctccccttcagt

SEQ ID NO: 319 - DNA, 20 bp, Artificial sequence
  Synthetic Oligonucleotide
agggaaggaggacagaatag

SEQ ID NO: 320 - DNA, 20 bp, Artificial sequence
  Synthetic Oligonucleotide
gaaatgaggtcaaatgtctg

SEQ ID NO: 321 - DNA, 20 bp, Artificial sequence
  Synthetic Oligonucleotide
ggagagtcagaaatgaggtc

SEQ ID NO: 322 - DNA, 20 bp, Artificial sequence
  Synthetic Oligonucleotide
gtagaaagtgggaggtgttg

SEQ ID NO: 323 - DNA, 20 bp, Artificial sequence
  Synthetic Oligonucleotide
tagaaagatctctgaagtgc

SEQ ID NO: 324 - DNA, 20 bp, Artificial sequence
  Synthetic Oligonucleotide
ctgctcctcaccccagtcct

SEQ ID NO: 325 - DNA, 20 bp, Artificial sequence
  Synthetic Oligonucleotide
ctactgggattctgtgctta

SEQ ID NO: 326 - DNA, 20 bp, Artificial sequence
  Synthetic Oligonucleotide
cccaaaaggccaaggaggga

SEQ ID NO: 327 - DNA, 20 bp, Artificial sequence
  Synthetic Oligonucleotide
tgaccacttggcatctcccc

SEQ ID NO: 328 - DNA, 20 bp, Artificial sequence
  Synthetic Oligonucleotide
cctgcaaggagaggagaagc

SEQ ID NO: 329 - DNA, 20 bp, Artificial sequence
  Synthetic Oligonucleotide
ctctcacctctgcaagtatt

SEQ ID NO: 330 - DNA, 20 bp, Artificial sequence
  Synthetic Oligonucleotide
ccccaaaaggccaaggaggg

SEQ ID NO: 331 - DNA, 20 bp, Artificial sequence
  Synthetic Oligonucleotide
gtcttccaagccatctttta

SEQ ID NO: 332 - DNA, 20 bp, Artificial sequence
  Synthetic Oligonucleotide
gttacaagtggacttaaggg

SEQ ID NO: 333 - DNA, 20 bp, Artificial sequence
  Synthetic Oligonucleotide
cccatgttgtgcaatcctgc

SEQ ID NO: 334 - DNA, 20 bp, Artificial sequence
  Synthetic Oligonucleotide
gaggtgggaagcatggagaa

SEQ ID NO: 335 - DNA, 20 bp, Artificial sequence
  Synthetic Oligonucleotide
tgctcccaccactgtcatct

SEQ ID NO: 336 - DNA, 20 bp, Artificial sequence
  Synthetic Oligonucleotide
aggcaggttactcacccaga

SEQ ID NO: 337 - DNA, 20 bp, Artificial sequence
  Synthetic Oligonucleotide
tactgggattctgtgcttac

SEQ ID NO: 338 - DNA, 20 bp, Artificial sequence
  Synthetic Oligonucleotide
gcctttcccagcctttcctc

SEQ ID NO: 339 - DNA, 20 bp, Artificial sequence
  Synthetic Oligonucleotide
gtgcaatcctgcagaagaga

SEQ ID NO: 340 - DNA, 20 bp, Artificial sequence
  Synthetic Oligonucleotide
acaggagagaggtcccttct

SEQ ID NO: 341 - DNA, 20 bp, Artificial sequence
  Synthetic Oligonucleotide
cccaaaaggagaaagggaaa

SEQ ID NO: 342 - DNA, 20 bp, Artificial sequence
  Synthetic Oligonucleotide
aagcccagggtaaatgctta

SEQ ID NO: 343 - DNA, 20 bp, Artificial sequence
  Synthetic Oligonucleotide
gatgaagcctggccccaaaa

SEQ ID NO: 344 - DNA, 20 bp, Artificial sequence
  Synthetic Oligonucleotide
tggcagagaaggagaatgtg

SEQ ID NO: 345 - DNA, 20 bp, Artificial sequence
  Synthetic Oligonucleotide
ttcccagcctttcctcaggg

SEQ ID NO: 346 - DNA, 20 bp, Artificial sequence
  Synthetic Oligonucleotide
ggcagagaaggagaatgtgc

SEQ ID NO: 347 - DNA, 20 bp, Artificial sequence
  Synthetic Oligonucleotide
acagtgccaggaaacaagaa

SEQ ID NO: 348 - DNA, 20 bp, Artificial sequence
  Synthetic Oligonucleotide
taggcaggttactcacccag

SEQ ID NO: 349 - DNA, 20 bp, Artificial sequence
  Synthetic Oligonucleotide
ttctcttgacttccagggct

SEQ ID NO: 350 - DNA, 20 bp, Artificial sequence
  Synthetic Oligonucleotide
cctgctcctcaccccagtcc

SEQ ID NO: 351 - DNA, 20 bp, Artificial sequence
  Synthetic Oligonucleotide
tcccactaacctccattgcc

SEQ ID NO: 352 - DNA, 20 bp, Artificial sequence
  Synthetic Oligonucleotide
ttccctttgaccacaaagtg

SEQ ID NO: 353 - DNA, 20 bp, Artificial sequence
  Synthetic Oligonucleotide
ctgggtcctaggcaggttac

SEQ ID NO: 354 - DNA, 20 bp, Artificial sequence
  Synthetic Oligonucleotide
tccaggcaactagagcttca

SEQ ID NO: 355 - DNA, 20 bp, Artificial sequence
  Synthetic Oligonucleotide
gcccatgttgtgcaatcctg

SEQ ID NO: 356 - DNA, 20 bp, Artificial sequence
  Synthetic Oligonucleotide
ggttcccactaacctccatt

SEQ ID NO: 357 - DNA, 20 bp, Artificial sequence
  Synthetic Oligonucleotide
aggtagagagcaagagttac

SEQ ID NO: 358 - DNA, 20 bp, Artificial sequence
  Synthetic Oligonucleotide
ccactaacctccattgccca

SEQ ID NO: 359 - DNA, 20 bp, Artificial sequence
  Synthetic Oligonucleotide
tcacaaaccaccatctctta

SEQ ID NO: 360 - DNA, 20 bp, Artificial sequence
  Synthetic Oligonucleotide
tactcacccagataatcctc

SEQ ID NO: 361 - DNA, 20 bp, Artificial sequence
  Synthetic Oligonucleotide
tgctcctcaccccagtcctc

SEQ ID NO: 362 - DNA, 20 bp, Artificial sequence
  Synthetic Oligonucleotide
tctcacagctgcctttctgt

SEQ ID NO: 363 - DNA, 20 bp, Artificial sequence
  Synthetic Oligonucleotide
gaaagggaggactcacttga

SEQ ID NO: 364 - DNA, 20 bp, Artificial sequence
  Synthetic Oligonucleotide
ccatcttttaaccccagaga

SEQ ID NO: 365 - DNA, 20 bp, Artificial sequence
  Synthetic Oligonucleotide
tcctcaccccagtcctccag

SEQ ID NO: 366 - DNA, 20 bp, Artificial sequence
  Synthetic Oligonucleotide
ctggcagagaaggagaatgt

SEQ ID NO: 367 - DNA, 20 bp, Artificial sequence
  Synthetic Oligonucleotide
tctccccagataggaaaggg

SEQ ID NO: 368 - DNA, 20 bp, Artificial sequence
  Synthetic Oligonucleotide
acttcagctgctcccaccac

SEQ ID NO: 369 - DNA, 20 bp, Artificial sequence
  Synthetic Oligonucleotide
gacagcaggaagggaaggtt

SEQ ID NO: 370 - DNA, 20 bp, Artificial sequence
  Synthetic Oligonucleotide
ggagacaaatgggcctataa

SEQ ID NO: 371 - DNA, 20 bp, Artificial sequence
  Synthetic Oligonucleotide
ctgctcccaccactgtcatc

SEQ ID NO: 372 - DNA, 20 bp, Artificial sequence
  Synthetic Oligonucleotide
aggaatgaagaaggctttcc

SEQ ID NO: 373 - DNA, 20 bp, Artificial sequence
  Synthetic Oligonucleotide
gggatctcatccttatcctc

SEQ ID NO: 374 - DNA, 20 bp, Artificial sequence
  Synthetic Oligonucleotide
gtgctgggtcctaggcaggt

SEQ ID NO: 375 - DNA, 20 bp, Artificial sequence
  Synthetic Oligonucleotide
caaaaggccaaggagggatg

SEQ ID NO: 376 - DNA, 20 bp, Artificial sequence
  Synthetic Oligonucleotide
ccatgctgaccacttggcat

SEQ ID NO: 377 - DNA, 20 bp, Artificial sequence
  Synthetic Oligonucleotide
ggaggctgggacaggagaga

SEQ ID NO: 378 - DNA, 20 bp, Artificial sequence
  Synthetic Oligonucleotide
ggagcagctcttcctctgga

SEQ ID NO: 379 - DNA, 20 bp, Artificial sequence
  Synthetic Oligonucleotide
tctcacctccgttgtcacag

SEQ ID NO: 380 - DNA, 20 bp, Artificial sequence
  Synthetic Oligonucleotide
cagtcctccagcctttccca

SEQ ID NO: 381 - DNA, 20 bp, Artificial sequence
  Synthetic Oligonucleotide
agtcctccagcctttcccag

SEQ ID NO: 382 - DNA, 20 bp, Artificial sequence
  Synthetic Oligonucleotide
tgaaggagtctgggagagtc

SEQ ID NO: 383 - DNA, 20 bp, Artificial sequence
  Synthetic Oligonucleotide
cagaatcacctgcaaggaga

SEQ ID NO: 384 - DNA, 20 bp, Artificial sequence
  Synthetic Oligonucleotide
taggaaagggaggactcact

SEQ ID NO: 385 - DNA, 20 bp, Artificial sequence
  Synthetic Oligonucleotide
accttggcaggaaggctccg

SEQ ID NO: 386 - DNA, 20 bp, Artificial sequence
  Synthetic Oligonucleotide
gagacaaatgggcctataaa

SEQ ID NO: 387 - DNA, 20 bp, Artificial sequence
  Synthetic Oligonucleotide
ctgaagagaaaggctgatga

SEQ ID NO: 388 - DNA, 20 bp, Artificial sequence
  Synthetic Oligonucleotide
aatgatcagggagctagtcc

SEQ ID NO: 389 - DNA, 20 bp, Artificial sequence
  Synthetic Oligonucleotide
cttagctgacctaaaggaat

SEQ ID NO: 390 - DNA, 20 bp, Artificial sequence
  Synthetic Oligonucleotide
tgggtatagtgttacaagtg

SEQ ID NO: 391 - DNA, 20 bp, Artificial sequence
  Synthetic Oligonucleotide
tgaagagaaaggctgatgaa

SEQ ID NO: 392 - DNA, 20 bp, Artificial sequence
  Synthetic Oligonucleotide
gtgttacaagtggacttaag

SEQ ID NO: 393 - DNA, 20 bp, Artificial sequence
  Synthetic Oligonucleotide
acctgtgggtgaggagaaca

SEQ ID NO: 394 - DNA, 20 bp, Artificial sequence
  Synthetic Oligonucleotide
tcacccagataatcctccct

SEQ ID NO: 395 - DNA, 20 bp, Artificial sequence
  Synthetic Oligonucleotide
tgttgtcgcagctgttttaa

SEQ ID NO: 396 - DNA, 20 bp, Artificial sequence
  Synthetic Oligonucleotide
tggtcacattcccttcccct

SEQ ID NO: 397 - DNA, 20 bp, Artificial sequence
  Synthetic Oligonucleotide
cctggtcacattcccttccc

SEQ ID NO: 398 - DNA, 20 bp, Artificial sequence
  Synthetic Oligonucleotide
tagacctggtcacattccct

SEQ ID NO: 399 - DNA, 20 bp, Artificial sequence
  Synthetic Oligonucleotide
cctagacctggtcacattcc

SEQ ID NO: 400 - DNA, 20 bp, Artificial sequence
  Synthetic Oligonucleotide
ccttccgagtcagctttttc

SEQ ID NO: 401 - DNA, 20 bp, Artificial sequence
  Synthetic Oligonucleotide
ctccttccgagtcagctttt

SEQ ID NO: 402 - DNA, 20 bp, Artificial sequence
  Synthetic Oligonucleotide
agacctccttccgagtcagc

SEQ ID NO: 403 - DNA, 20 bp, Artificial sequence
  Synthetic Oligonucleotide
gtagacctccttccgagtca

SEQ ID NO: 404 - DNA, 20 bp, Artificial sequence
  Synthetic Oligonucleotide
tttgccgcttctggtttttg

SEQ ID NO: 405 - DNA, 20 bp, Artificial sequence
  Synthetic Oligonucleotide
cttttgccgcttctggtttt

SEQ ID NO: 406 - DNA, 20 bp, Artificial sequence
  Synthetic Oligonucleotide
cctgcttttgccgcttctgg

SEQ ID NO: 407 - DNA, 20 bp, Artificial sequence
  Synthetic Oligonucleotide
tacctgcttttgccgcttct

SEQ ID NO: 408 - DNA, 20 bp, Artificial sequence
  Synthetic Oligonucleotide
agaaaacccaaatcctcatc

SEQ ID NO: 409 - DNA, 20 bp, Artificial sequence
  Synthetic Oligonucleotide
tagaaaacccaaatcctcat

SEQ ID NO: 410 - DNA, 20 bp, Artificial sequence
  Synthetic Oligonucleotide
atagaaaacccaaatcctca

SEQ ID NO: 411 - DNA, 20 bp, Artificial sequence
  Synthetic Oligonucleotide
tatagaaaacccaaatcctc

SEQ ID NO: 412 - DNA, 20 bp, Artificial sequence
  Synthetic Oligonucleotide
ttatagaaaacccaaatcct

SEQ ID NO: 413 - DNA, 20 bp, Artificial sequence
  Synthetic Oligonucleotide
cttatagaaaacccaaatcc

SEQ ID NO: 414 - DNA, 20 bp, Artificial sequence
  Synthetic Oligonucleotide
ccttatagaaaacccaaatc

SEQ ID NO: 415 - DNA, 20 bp, Artificial sequence
  Synthetic Oligonucleotide
cccttatagaaaacccaaat

SEQ ID NO: 416 - DNA, 20 bp, Artificial sequence
  Synthetic Oligonucleotide
ccccttatagaaaacccaaa

SEQ ID NO: 417 - DNA, 20 bp, Artificial sequence
  Synthetic Oligonucleotide
accccttatagaaaacccaa

SEQ ID NO: 418 - DNA, 20 bp, Artificial sequence
  Synthetic Oligonucleotide
aaccccttatagaaaaccca

SEQ ID NO: 419 - DNA, 20 bp, Artificial sequence
  Synthetic Oligonucleotide
aaaccccttatagaaaaccc

SEQ ID NO: 420 - DNA, 20 bp, Artificial sequence
  Synthetic Oligonucleotide
gaaaccccttatagaaaacc

SEQ ID NO: 421 - DNA, 20 bp, Artificial sequence
  Synthetic Oligonucleotide
ggaaaccccttatagaaaac

SEQ ID NO: 422 - DNA, 20 bp, Artificial sequence
  Synthetic Oligonucleotide
aggaaaccccttatagaaaa

SEQ ID NO: 423 - DNA, 20 bp, Artificial sequence
  Synthetic Oligonucleotide
caggaaaccccttatagaaa

SEQ ID NO: 424 - DNA, 20 bp, Artificial sequence
  Synthetic Oligonucleotide
gcaggaaaccccttatagaa

SEQ ID NO: 425 - DNA, 20 bp, Artificial sequence
  Synthetic Oligonucleotide
agcaggaaaccccttataga

SEQ ID NO: 426 - DNA, 20 bp, Artificial sequence
  Synthetic Oligonucleotide
cagcaggaaaccccttatag

SEQ ID NO: 427 - DNA, 20 bp, Artificial sequence
  Synthetic Oligonucleotide
ccagcaggaaaccccttata

SEQ ID NO: 428 - DNA, 20 bp, Artificial sequence
  Synthetic Oligonucleotide
tccagcaggaaaccccttat

SEQ ID NO: 429 - DNA, 20 bp, Artificial sequence
  Synthetic Oligonucleotide
tgtccagcaggaaacccctt

SEQ ID NO: 430 - DNA, 20 bp, Artificial sequence
  Synthetic Oligonucleotide
ctgtccagcaggaaacccct

SEQ ID NO: 431 - DNA, 20 bp, Artificial sequence
  Synthetic Oligonucleotide
cctgtccagcaggaaacccc

SEQ ID NO: 432 - DNA, 20 bp, Artificial sequence
  Synthetic Oligonucleotide
ccctgtccagcaggaaaccc

SEQ ID NO: 433 - DNA, 20 bp, Artificial sequence
  Synthetic Oligonucleotide
cccctgtccagcaggaaacc

SEQ ID NO: 434 - DNA, 20 bp, Artificial sequence
  Synthetic Oligonucleotide
cgcccctgtccagcaggaaa

SEQ ID NO: 435 - DNA, 20 bp, Artificial sequence
  Synthetic Oligonucleotide
acgcccctgtccagcaggaa

SEQ ID NO: 436 - DNA, 20 bp, Artificial sequence
  Synthetic Oligonucleotide
cacgcccctgtccagcagga

SEQ ID NO: 437 - DNA, 20 bp, Artificial sequence
  Synthetic Oligonucleotide
ccacgcccctgtccagcagg

SEQ ID NO: 438 - DNA, 20 bp, Artificial sequence
  Synthetic Oligonucleotide
cccacgcccctgtccagcag

SEQ ID NO: 439 - DNA, 20 bp, Artificial sequence
  Synthetic Oligonucleotide
tcccacgcccctgtccagca

SEQ ID NO: 440 - DNA, 20 bp, Artificial sequence
  Synthetic Oligonucleotide
atcccacgcccctgtccagc

SEQ ID NO: 441 - DNA, 20 bp, Artificial sequence
  Synthetic Oligonucleotide
aatcccacgcccctgtccag

SEQ ID NO: 442 - DNA, 20 bp, Artificial sequence
  Synthetic Oligonucleotide
caatcccacgcccctgtcca

SEQ ID NO: 443 - DNA, 20 bp, Artificial sequence
  Synthetic Oligonucleotide
tcaatcccacgcccctgtcc

SEQ ID NO: 444 - DNA, 20 bp, Artificial sequence
  Synthetic Oligonucleotide
ttcaatcccacgcccctgtc

SEQ ID NO: 445 - DNA, 20 bp, Artificial sequence
  Synthetic Oligonucleotide
attcaatcccacgcccctgt

SEQ ID NO: 446 - DNA, 20 bp, Artificial sequence
  Synthetic Oligonucleotide
aattcaatcccacgcccctg

SEQ ID NO: 447 - DNA, 20 bp, Artificial sequence
  Synthetic Oligonucleotide
taattcaatcccacgcccct

SEQ ID NO: 448 - DNA, 20 bp, Artificial sequence
  Synthetic Oligonucleotide
ttaattcaatcccacgcccc

SEQ ID NO: 449 - DNA, 20 bp, Artificial sequence
  Synthetic Oligonucleotide
tttaattcaatcccacgccc

SEQ ID NO: 450 - DNA, 20 bp, Artificial sequence
  Synthetic Oligonucleotide
ttttaattcaatcccacgcc

SEQ ID NO: 451 - DNA, 20 bp, Artificial sequence
  Synthetic Oligonucleotide
gttttaattcaatcccacgc

SEQ ID NO: 452 - DNA, 20 bp, Artificial sequence
  Synthetic Oligonucleotide
tgttttaattcaatcccacg

SEQ ID NO: 453 - DNA, 20 bp, Artificial sequence
  Synthetic Oligonucleotide
ctgttttaattcaatcccac

SEQ ID NO: 454 - DNA, 20 bp, Artificial sequence
  Synthetic Oligonucleotide
gctgttttaattcaatccca

SEQ ID NO: 455 - DNA, 20 bp, Artificial sequence
  Synthetic Oligonucleotide
cagctgttttaattcaatcc

SEQ ID NO: 456 - DNA, 20 bp, Artificial sequence
  Synthetic Oligonucleotide
gcagctgttttaattcaatc

SEQ ID NO: 457 - DNA, 20 bp, Artificial sequence
  Synthetic Oligonucleotide
cgcagctgttttaattcaat

SEQ ID NO: 458 - DNA, 20 bp, Artificial sequence
  Synthetic Oligonucleotide
tcgcagctgttttaattcaa

SEQ ID NO: 459 - DNA, 20 bp, Artificial sequence
  Synthetic Oligonucleotide
tgtcgcagctgttttaattc

SEQ ID NO: 460 - DNA, 20 bp, Artificial sequence
  Synthetic Oligonucleotide
ttgtcgcagctgttttaatt

SEQ ID NO: 461 - DNA, 20 bp, Artificial sequence
  Synthetic Oligonucleotide
gttgtcgcagctgttttaat

SEQ ID NO: 462 - DNA, 20 bp, Artificial sequence
  Synthetic Oligonucleotide
ttgttgtcgcagctgtttta

SEQ ID NO: 463 - DNA, 20 bp, Artificial sequence
  Synthetic Oligonucleotide
tttgttgtcgcagctgtttt

SEQ ID NO: 464 - DNA, 20 bp, Artificial sequence
  Synthetic Oligonucleotide
ttttgttgtcgcagctgttt

SEQ ID NO: 465 - DNA, 20 bp, Artificial sequence
  Synthetic Oligonucleotide
tttttgttgtcgcagctgtt

SEQ ID NO: 466 - DNA, 20 bp, Artificial sequence
  Synthetic Oligonucleotide
ggatccagctcactcccctg

SEQ ID NO: 467 - DNA, 20 bp, Artificial sequence
  Synthetic Oligonucleotide
aaataaggatccagctcact

SEQ ID NO: 468 - DNA, 20 bp, Artificial sequence
  Synthetic Oligonucleotide
gaccagaaataaggatccag

SEQ ID NO: 469 - DNA, 20 bp, Artificial sequence
  Synthetic Oligonucleotide
cttagggaccagaaataagg

SEQ ID NO: 470 - DNA, 20 bp, Artificial sequence
  Synthetic Oligonucleotide
cacccacttagggaccagaa

SEQ ID NO: 471 - DNA, 20 bp, Artificial sequence
  Synthetic Oligonucleotide
accacccacttagggaccag

SEQ ID NO: 472 - DNA, 20 bp, Artificial sequence
  Synthetic Oligonucleotide
aggtccaggactctcccctt

SEQ ID NO: 473 - DNA, 20 bp, Artificial sequence
  Synthetic Oligonucleotide
aaggtccaggactctcccct

SEQ ID NO: 474 - DNA, 20 bp, Artificial sequence
  Synthetic Oligonucleotide
aaactgcagaagtcccaccc

SEQ ID NO: 475 - DNA, 20 bp, Artificial sequence
  Synthetic Oligonucleotide
ggagggccccgctgagctgc

SEQ ID NO: 476 - DNA, 20 bp, Artificial sequence
  Synthetic Oligonucleotide
tcccggaacatccaagcggg

SEQ ID NO: 477 - DNA, 20 bp, Artificial sequence
  Synthetic Oligonucleotide
catcactttcccggaacatc

SEQ ID NO: 478 - DNA, 20 bp, Artificial sequence
  Synthetic Oligonucleotide
ctggtcacattcccttcccc

SEQ ID NO: 479 - DNA, 20 bp, Artificial sequence
  Synthetic Oligonucleotide
ctagacctggtcacattccc

SEQ ID NO: 480 - DNA, 20 bp, Artificial sequence
  Synthetic Oligonucleotide
ggagtggtggtcacacctcc

SEQ ID NO: 481 - DNA, 20 bp, Artificial sequence
  Synthetic Oligonucleotide
accccctccagagagcagga

SEQ ID NO: 482 - DNA, 20 bp, Artificial sequence
  Synthetic Oligonucleotide
atctctaccccctccagaga

SEQ ID NO: 483 - DNA, 20 bp, Artificial sequence
  Synthetic Oligonucleotide
ggtacgggtagaagccagaa

SEQ ID NO: 484 - DNA, 20 bp, Artificial sequence
  Synthetic Oligonucleotide
ggagagtgtaaccgtcatag

SEQ ID NO: 485 - DNA, 20 bp, Artificial sequence
  Synthetic Oligonucleotide
tgcgattggcagagccccgg

SEQ ID NO: 486 - DNA, 20 bp, Artificial sequence
  Synthetic Oligonucleotide
ggcaggtgcgattggcagag

SEQ ID NO: 487 - DNA, 20 bp, Artificial sequence
  Synthetic Oligonucleotide
ggccattcacttggcaggtg

SEQ ID NO: 488 - DNA, 20 bp, Artificial sequence
  Synthetic Oligonucleotide
ttgtcacagatcgctgtctg

SEQ ID NO: 489 - DNA, 20 bp, Artificial sequence
  Synthetic Oligonucleotide
aaggagtcttggcaggaagg

SEQ ID NO: 490 - DNA, 20 bp, Artificial sequence
  Synthetic Oligonucleotide
gtacatgaaggagtcttggc

SEQ ID NO: 491 - DNA, 20 bp, Artificial sequence
  Synthetic Oligonucleotide
aagcttcggccacctcttga

SEQ ID NO: 492 - DNA, 20 bp, Artificial sequence
  Synthetic Oligonucleotide
ccatctagcaccaggtagat

SEQ ID NO: 493 - DNA, 20 bp, Artificial sequence
  Synthetic Oligonucleotide
ggccccaatgctgtctgatc

SEQ ID NO: 494 - DNA, 20 bp, Artificial sequence
  Synthetic Oligonucleotide
aattaagttgactagacact

SEQ ID NO: 495 - DNA, 20 bp, Artificial sequence
  Synthetic Oligonucleotide
tgccaccttctcaattaagt

SEQ ID NO: 496 - DNA, 20 bp, Artificial sequence
  Synthetic Oligonucleotide
taacttgccaccttctcaat

SEQ ID NO: 497 - DNA, 20 bp, Artificial sequence
  Synthetic Oligonucleotide
cataacttgccaccttctca

SEQ ID NO: 498 - DNA, 20 bp, Artificial sequence
  Synthetic Oligonucleotide
acaccataacttgccacctt

SEQ ID NO: 499 - DNA, 20 bp, Artificial sequence
  Synthetic Oligonucleotide
tcacaccataacttgccacc

SEQ ID NO: 500 - DNA, 20 bp, Artificial sequence
  Synthetic Oligonucleotide
tagtccctgacttcaacttg

SEQ ID NO: 501 - DNA, 20 bp, Artificial sequence
  Synthetic Oligonucleotide
tggtgttagtccctgacttc

SEQ ID NO: 502 - DNA, 20 bp, Artificial sequence
  Synthetic Oligonucleotide
gcggttccagccttcaggag

SEQ ID NO: 503 - DNA, 20 bp, Artificial sequence
  Synthetic Oligonucleotide
tcatgaggatgatgacatgg

SEQ ID NO: 504 - DNA, 20 bp, Artificial sequence
  Synthetic Oligonucleotide
ccgcccatgttgtgcaatcc

SEQ ID NO: 505 - DNA, 20 bp, Artificial sequence
  Synthetic Oligonucleotide
gtaattgggtccccgcccat

SEQ ID NO: 506 - DNA, 20 bp, Artificial sequence
  Synthetic Oligonucleotide
aagtcccggatctcatcaat

SEQ ID NO: 507 - DNA, 20 bp, Artificial sequence
  Synthetic Oligonucleotide
aacacatagacatccagata

SEQ ID NO: 508 - DNA, 20 bp, Artificial sequence
  Synthetic Oligonucleotide
caaagcattgatgttcactt

SEQ ID NO: 509 - DNA, 20 bp, Artificial sequence
  Synthetic Oligonucleotide
tttgaacacatgttgctcat

SEQ ID NO: 510 - DNA, 20 bp, Artificial sequence
  Synthetic Oligonucleotide
cttccaggttttccatatcc

SEQ ID NO: 511 - DNA, 20 bp, Artificial sequence
  Synthetic Oligonucleotide
tcttccaggttttccatatc

SEQ ID NO: 512 - DNA, 20 bp, Artificial sequence
  Synthetic Oligonucleotide
agactcagagactggctttc

SEQ ID NO: 513 - DNA, 20 bp, Artificial sequence
  Synthetic Oligonucleotide
gcctgccatggttgcttgtg

SEQ ID NO: 514 - DNA, 20 bp, Artificial sequence
  Synthetic Oligonucleotide
tgactgagatcttggcctgc

SEQ ID NO: 515 - DNA, 20 bp, Artificial sequence
  Synthetic Oligonucleotide
ttctatctccaggtcccgct

SEQ ID NO: 516 - DNA, 20 bp, Artificial sequence
  Synthetic Oligonucleotide
agtcataaaattcaggaatt

SEQ ID NO: 517 - DNA, 20 bp, Artificial sequence
  Synthetic Oligonucleotide
cgagttgttccctcggtgca

SEQ ID NO: 518 - DNA, 20 bp, Artificial sequence
  Synthetic Oligonucleotide
agcctcaaagctcgagttgt

SEQ ID NO: 519 - DNA, 20 bp, Artificial sequence
  Synthetic Oligonucleotide
ggaggaagcctcaaagctcg

SEQ ID NO: 520 - DNA, 20 bp, Artificial sequence
  Synthetic Oligonucleotide
gtagttggaggaagcctcaa

SEQ ID NO: 521 - DNA, 20 bp, Artificial sequence
  Synthetic Oligonucleotide
caagtggtagttggaggaag

SEQ ID NO: 522 - DNA, 20 bp, Artificial sequence
  Synthetic Oligonucleotide
tcctcagacacaaacagagc

SEQ ID NO: 523 - DNA, 20 bp, Artificial sequence
  Synthetic Oligonucleotide
ttctcctcctcagacacaaa

SEQ ID NO: 524 - DNA, 20 bp, Artificial sequence
  Synthetic Oligonucleotide
tagacctccttccgagtcag

SEQ ID NO: 525 - DNA, 20 bp, Artificial sequence
  Synthetic Oligonucleotide
ttgatgtagacctccttccg

SEQ ID NO: 526 - DNA, 20 bp, Artificial sequence
  Synthetic Oligonucleotide
ctttcttatccccattcttg

SEQ ID NO: 527 - DNA, 20 bp, Artificial sequence
  Synthetic Oligonucleotide
gcctttcttatccccattct

SEQ ID NO: 528 - DNA, 20 bp, Artificial sequence
  Synthetic Oligonucleotide
agctgcctttcttatcccca

SEQ ID NO: 529 - DNA, 20 bp, Artificial sequence
  Synthetic Oligonucleotide
cagctgcctttcttatcccc

SEQ ID NO: 530 - DNA, 20 bp, Artificial sequence
  Synthetic Oligonucleotide
acagctgcctttcttatccc

SEQ ID NO: 531 - DNA, 20 bp, Artificial sequence
  Synthetic Oligonucleotide
gcatctctctcacagctgcc

SEQ ID NO: 532 - DNA, 20 bp, Artificial sequence
  Synthetic Oligonucleotide
agatgtccttgactttgtca

SEQ ID NO: 533 - DNA, 20 bp, Artificial sequence
  Synthetic Oligonucleotide
cagcatagggactcactcct

SEQ ID NO: 534 - DNA, 20 bp, Artificial sequence
  Synthetic Oligonucleotide
ccgccagaatcacctctgca

SEQ ID NO: 535 - DNA, 20 bp, Artificial sequence
  Synthetic Oligonucleotide
tgaatgaaacgacttctctt

SEQ ID NO: 536 - DNA, 20 bp, Artificial sequence
  Synthetic Oligonucleotide
acatccactactccccagct

SEQ ID NO: 537 - DNA, 20 bp, Artificial sequence
  Synthetic Oligonucleotide
cgcttctggtttttgcagac

SEQ ID NO: 538 - DNA, 20 bp, Artificial sequence
  Synthetic Oligonucleotide
ttttgccgcttctggttttt

SEQ ID NO: 539 - DNA, 20 bp, Artificial sequence
  Synthetic Oligonucleotide
gcaggtacctgcttttgccg

SEQ ID NO: 540 - DNA, 20 bp, Artificial sequence
  Synthetic Oligonucleotide
tcttggagtttctccttcag

SEQ ID NO: 541 - DNA, 16 bp, Artificial sequence
  Synthetic Oligonucleotide
ggaacatccaagcggg

SEQ ID NO: 542 - DNA, 16 bp, Artificial sequence
  Synthetic Oligonucleotide
tggtcacattcccttc

SEQ ID NO: 543 - DNA, 16 bp, Artificial sequence
  Synthetic Oligonucleotide
cctggtcacattccct

SEQ ID NO: 544 - DNA, 16 bp, Artificial sequence
  Synthetic Oligonucleotide
gacctggtcacattcc

SEQ ID NO: 545 - DNA, 16 bp, Artificial sequence
  Synthetic Oligonucleotide
taacttgccaccttct

SEQ ID NO: 546 - DNA, 16 bp, Artificial sequence
  Synthetic Oligonucleotide
cataacttgccacctt

SEQ ID NO: 547 - DNA, 16 bp, Artificial sequence
  Synthetic Oligonucleotide
accataacttgccacc

SEQ ID NO: 548 - DNA, 16 bp, Artificial sequence
  Synthetic Oligonucleotide
ccttccgagtcagctt

SEQ ID NO: 549 - DNA, 16 bp, Artificial sequence
  Synthetic Oligonucleotide
ctccttccgagtcagc

SEQ ID NO: 550 - DNA, 16 bp, Artificial sequence
  Synthetic Oligonucleotide
acctccttccgagtca

SEQ ID NO: 551 - DNA, 16 bp, Artificial sequence
  Synthetic Oligonucleotide
ctttcttatccccatt

SEQ ID NO: 552 - DNA, 16 bp, Artificial sequence
  Synthetic Oligonucleotide
gcctttcttatcccca

SEQ ID NO: 553 - DNA, 16 bp, Artificial sequence
  Synthetic Oligonucleotide
ctgcctttcttatccc

SEQ ID NO: 554 - DNA, 16 bp, Artificial sequence
  Synthetic Oligonucleotide
tttgccgcttctggtt

SEQ ID NO: 555 - DNA, 16 bp, Artificial sequence
  Synthetic Oligonucleotide
cttttgccgcttctgg

SEQ ID NO: 556 - DNA, 16 bp, Artificial sequence
  Synthetic Oligonucleotide
tgcttttgccgcttct

SEQ ID NO: 557 - DNA, 16 bp, Artificial sequence
  Synthetic Oligonucleotide
aaacccaaatcctcat

SEQ ID NO: 558 - DNA, 16 bp, Artificial sequence
  Synthetic Oligonucleotide
gaaaacccaaatcctc

SEQ ID NO: 559 - DNA, 16 bp, Artificial sequence
  Synthetic Oligonucleotide
tagaaaacccaaatcc

SEQ ID NO: 560 - DNA, 16 bp, Artificial sequence
  Synthetic Oligonucleotide
atagaaaacccaaatc

SEQ ID NO: 561 - DNA, 16 bp, Artificial sequence
  Synthetic Oligonucleotide
cttatagaaaacccaa

SEQ ID NO: 562 - DNA, 16 bp, Artificial sequence
  Synthetic Oligonucleotide
ccttatagaaaaccca

SEQ ID NO: 563 - DNA, 16 bp, Artificial sequence
  Synthetic Oligonucleotide
cccttatagaaaaccc

SEQ ID NO: 564 - DNA, 16 bp, Artificial sequence
  Synthetic Oligonucleotide
ccccttatagaaaacc

SEQ ID NO: 565 - DNA, 16 bp, Artificial sequence
  Synthetic Oligonucleotide
accccttatagaaaac

SEQ ID NO: 566 - DNA, 16 bp, Artificial sequence
  Synthetic Oligonucleotide
aaccccttatagaaaa

SEQ ID NO: 567 - DNA, 16 bp, Artificial sequence
  Synthetic Oligonucleotide
aaaccccttatagaaa

SEQ ID NO: 568 - DNA, 16 bp, Artificial sequence
  Synthetic Oligonucleotide
gaaaccccttatagaa

SEQ ID NO: 569 - DNA, 16 bp, Artificial sequence
  Synthetic Oligonucleotide
ggaaaccccttataga

SEQ ID NO: 570 - DNA, 16 bp, Artificial sequence
  Synthetic Oligonucleotide
aggaaaccccttatag

SEQ ID NO: 571 - DNA, 16 bp, Artificial sequence
  Synthetic Oligonucleotide
caggaaaccccttata

SEQ ID NO: 572 - DNA, 16 bp, Artificial sequence
  Synthetic Oligonucleotide
gcaggaaaccccttat

SEQ ID NO: 573 - DNA, 16 bp, Artificial sequence
  Synthetic Oligonucleotide
agcaggaaacccctta

SEQ ID NO: 574 - DNA, 16 bp, Artificial sequence
  Synthetic Oligonucleotide
cagcaggaaacccctt

SEQ ID NO: 575 - DNA, 16 bp, Artificial sequence
  Synthetic Oligonucleotide
ccagcaggaaacccct

SEQ ID NO: 576 - DNA, 16 bp, Artificial sequence
  Synthetic Oligonucleotide
tccagcaggaaacccc

SEQ ID NO: 577 - DNA, 16 bp, Artificial sequence
  Synthetic Oligonucleotide
gtccagcaggaaaccc

SEQ ID NO: 578 - DNA, 16 bp, Artificial sequence
  Synthetic Oligonucleotide
tgtccagcaggaaacc

SEQ ID NO: 579 - DNA, 16 bp, Artificial sequence
  Synthetic Oligonucleotide
ctgtccagcaggaaac

SEQ ID NO: 580 - DNA, 16 bp, Artificial sequence
  Synthetic Oligonucleotide
cctgtccagcaggaaa

SEQ ID NO: 581 - DNA, 16 bp, Artificial sequence
  Synthetic Oligonucleotide
ccctgtccagcaggaa

SEQ ID NO: 582 - DNA, 16 bp, Artificial sequence
  Synthetic Oligonucleotide
cccctgtccagcagga

SEQ ID NO: 583 - DNA, 16 bp, Artificial sequence
  Synthetic Oligonucleotide
gcccctgtccagcagg

SEQ ID NO: 584 - DNA, 16 bp, Artificial sequence
  Synthetic Oligonucleotide
cgcccctgtccagcag

SEQ ID NO: 585 - DNA, 16 bp, Artificial sequence
  Synthetic Oligonucleotide
acgcccctgtccagca

SEQ ID NO: 586 - DNA, 16 bp, Artificial sequence
  Synthetic Oligonucleotide
cacgcccctgtccagc

SEQ ID NO: 587 - DNA, 16 bp, Artificial sequence
  Synthetic Oligonucleotide
ccacgcccctgtccag

SEQ ID NO: 588 - DNA, 16 bp, Artificial sequence
  Synthetic Oligonucleotide
cccacgcccctgtcca

SEQ ID NO: 589 - DNA, 16 bp, Artificial sequence
  Synthetic Oligonucleotide
tcccacgcccctgtcc

SEQ ID NO: 590 - DNA, 16 bp, Artificial sequence
  Synthetic Oligonucleotide
atcccacgcccctgtc

SEQ ID NO: 591 - DNA, 16 bp, Artificial sequence
  Synthetic Oligonucleotide
aatcccacgcccctgt

SEQ ID NO: 592 - DNA, 16 bp, Artificial sequence
  Synthetic Oligonucleotide
caatcccacgcccctg

SEQ ID NO: 593 - DNA, 16 bp, Artificial sequence
  Synthetic Oligonucleotide
tcaatcccacgcccct

SEQ ID NO: 594 - DNA, 16 bp, Artificial sequence
  Synthetic Oligonucleotide
ttcaatcccacgcccc

SEQ ID NO: 595 - DNA, 16 bp, Artificial sequence
  Synthetic Oligonucleotide
attcaatcccacgccc

SEQ ID NO: 596 - DNA, 16 bp, Artificial sequence
  Synthetic Oligonucleotide
aattcaatcccacgcc

SEQ ID NO: 597 - DNA, 16 bp, Artificial sequence
  Synthetic Oligonucleotide
taattcaatcccacgc

SEQ ID NO: 598 - DNA, 16 bp, Artificial sequence
  Synthetic Oligonucleotide
ttaattcaatcccacg

SEQ ID NO: 599 - DNA, 16 bp, Artificial sequence
  Synthetic Oligonucleotide
tttaattcaatcccac

SEQ ID NO: 600 - DNA, 16 bp, Artificial sequence
  Synthetic Oligonucleotide
ttttaattcaatccca

SEQ ID NO: 601 - DNA, 16 bp, Artificial sequence
  Synthetic Oligonucleotide
gttttaattcaatccc

SEQ ID NO: 602 - DNA, 16 bp, Artificial sequence
  Synthetic Oligonucleotide
tgttttaattcaatcc

SEQ ID NO: 603 - DNA, 16 bp, Artificial sequence
  Synthetic Oligonucleotide
ctgttttaattcaatc

SEQ ID NO: 604 - DNA, 16 bp, Artificial sequence
  Synthetic Oligonucleotide
gctgttttaattcaat

SEQ ID NO: 605 - DNA, 16 bp, Artificial sequence
  Synthetic Oligonucleotide
agctgttttaattcaa

SEQ ID NO: 606 - DNA, 16 bp, Artificial sequence
  Synthetic Oligonucleotide
cagctgttttaattca

SEQ ID NO: 607 - DNA, 16 bp, Artificial sequence
  Synthetic Oligonucleotide
gcagctgttttaattc

SEQ ID NO: 608 - DNA, 16 bp, Artificial sequence
  Synthetic Oligonucleotide
cgcagctgttttaatt

SEQ ID NO: 609 - DNA, 16 bp, Artificial sequence
  Synthetic Oligonucleotide
tcgcagctgttttaat

SEQ ID NO: 610 - DNA, 16 bp, Artificial sequence
  Synthetic Oligonucleotide
gtcgcagctgttttaa

SEQ ID NO: 611 - DNA, 16 bp, Artificial sequence
  Synthetic Oligonucleotide
tgtcgcagctgtttta

SEQ ID NO: 612 - DNA, 16 bp, Artificial sequence
  Synthetic Oligonucleotide
ttgtcgcagctgtttt

SEQ ID NO: 613 - DNA, 16 bp, Artificial sequence
  Synthetic Oligonucleotide
gttgtcgcagctgttt

SEQ ID NO: 614 - DNA, 16 bp, Artificial sequence
  Synthetic Oligonucleotide
tgttgtcgcagctgtt

SEQ ID NO: 615 - DNA, 16 bp, Artificial sequence
  Synthetic Oligonucleotide
ttgttgtcgcagctgt

SEQ ID NO: 616 - DNA, 16 bp, Artificial sequence
  Synthetic Oligonucleotide
tttgttgtcgcagctg

SEQ ID NO: 617 - DNA, 16 bp, Artificial sequence
  Synthetic Oligonucleotide
ttttgttgtcgcagct

SEQ ID NO: 618 - DNA, 16 bp, Artificial sequence
  Synthetic Oligonucleotide
tttttgttgtcgcagc

SEQ ID NO: 619 - DNA, 17 bp, Artificial sequence
  Synthetic Oligonucleotide
gaaaacccaaatcctca

SEQ ID NO: 620 - DNA, 17 bp, Artificial sequence
  Synthetic Oligonucleotide
agaaaacccaaatcctc

SEQ ID NO: 621 - DNA, 17 bp, Artificial sequence
  Synthetic Oligonucleotide
tagaaaacccaaatcct

SEQ ID NO: 622 - DNA, 17 bp, Artificial sequence
  Synthetic Oligonucleotide
atagaaaacccaaatcc

SEQ ID NO: 623 - DNA, 17 bp, Artificial sequence
  Synthetic Oligonucleotide
ttatagaaaacccaaat

SEQ ID NO: 624 - DNA, 17 bp, Artificial sequence
  Synthetic Oligonucleotide
cttatagaaaacccaaa

SEQ ID NO: 625 - DNA, 17 bp, Artificial sequence
  Synthetic Oligonucleotide
ccttatagaaaacccaa

SEQ ID NO: 626 - DNA, 17 bp, Artificial sequence
  Synthetic Oligonucleotide
cccttatagaaaaccca

SEQ ID NO: 627 - DNA, 17 bp, Artificial sequence
  Synthetic Oligonucleotide
ccccttatagaaaaccc

SEQ ID NO: 628 - DNA, 17 bp, Artificial sequence
  Synthetic Oligonucleotide
accccttatagaaaacc

SEQ ID NO: 629 - DNA, 17 bp, Artificial sequence
  Synthetic Oligonucleotide
aaccccttatagaaaac

SEQ ID NO: 630 - DNA, 17 bp, Artificial sequence
  Synthetic Oligonucleotide
aaaccccttatagaaaa

SEQ ID NO: 631 - DNA, 17 bp, Artificial sequence
  Synthetic Oligonucleotide
gaaaccccttatagaaa

SEQ ID NO: 632 - DNA, 17 bp, Artificial sequence
  Synthetic Oligonucleotide
ggaaaccccttatagaa

SEQ ID NO: 633 - DNA, 17 bp, Artificial sequence
  Synthetic Oligonucleotide
aggaaaccccttataga

SEQ ID NO: 634 - DNA, 17 bp, Artificial sequence
  Synthetic Oligonucleotide
caggaaaccccttatag

SEQ ID NO: 635 - DNA, 17 bp, Artificial sequence
  Synthetic Oligonucleotide
gcaggaaaccccttata

SEQ ID NO: 636 - DNA, 17 bp, Artificial sequence
  Synthetic Oligonucleotide
agcaggaaaccccttat

SEQ ID NO: 637 - DNA, 17 bp, Artificial sequence
  Synthetic Oligonucleotide
cagcaggaaacccctta

SEQ ID NO: 638 - DNA, 17 bp, Artificial sequence
  Synthetic Oligonucleotide
ccagcaggaaacccctt

SEQ ID NO: 639 - DNA, 17 bp, Artificial sequence
  Synthetic Oligonucleotide
tccagcaggaaacccct

SEQ ID NO: 640 - DNA, 17 bp, Artificial sequence
  Synthetic Oligonucleotide
gtccagcaggaaacccc

SEQ ID NO: 641 - DNA, 17 bp, Artificial sequence
  Synthetic Oligonucleotide
tgtccagcaggaaaccc

SEQ ID NO: 642 - DNA, 17 bp, Artificial sequence
  Synthetic Oligonucleotide
ctgtccagcaggaaacc

SEQ ID NO: 643 - DNA, 17 bp, Artificial sequence
  Synthetic Oligonucleotide
cctgtccagcaggaaac

SEQ ID NO: 644 - DNA, 17 bp, Artificial sequence
  Synthetic Oligonucleotide
ccctgtccagcaggaaa

SEQ ID NO: 645 - DNA, 17 bp, Artificial sequence
  Synthetic Oligonucleotide
gcccctgtccagcagga

SEQ ID NO: 646 - DNA, 17 bp, Artificial sequence
  Synthetic Oligonucleotide
cgcccctgtccagcagg

SEQ ID NO: 647 - DNA, 17 bp, Artificial sequence
  Synthetic Oligonucleotide
acgcccctgtccagcag

SEQ ID NO: 648 - DNA, 17 bp, Artificial sequence
  Synthetic Oligonucleotide
cacgcccctgtccagca

SEQ ID NO: 649 - DNA, 17 bp, Artificial sequence
  Synthetic Oligonucleotide
ccacgcccctgtccagc

SEQ ID NO: 650 - DNA, 17 bp, Artificial sequence
  Synthetic Oligonucleotide
cccacgcccctgtccag

SEQ ID NO: 651 - DNA, 17 bp, Artificial sequence
  Synthetic Oligonucleotide
tcccacgcccctgtcca

SEQ ID NO: 652 - DNA, 17 bp, Artificial sequence
  Synthetic Oligonucleotide
atcccacgcccctgtcc

SEQ ID NO: 653 - DNA, 17 bp, Artificial sequence
  Synthetic Oligonucleotide
aatcccacgcccctgtc

SEQ ID NO: 654 - DNA, 17 bp, Artificial sequence
  Synthetic Oligonucleotide
caatcccacgcccctgt

SEQ ID NO: 655 - DNA, 17 bp, Artificial sequence
  Synthetic Oligonucleotide
tcaatcccacgcccctg

SEQ ID NO: 656 - DNA, 17 bp, Artificial sequence
  Synthetic Oligonucleotide
ttcaatcccacgcccct

SEQ ID NO: 657 - DNA, 17 bp, Artificial sequence
  Synthetic Oligonucleotide
attcaatcccacgcccc

SEQ ID NO: 658 - DNA, 17 bp, Artificial sequence
  Synthetic Oligonucleotide
aattcaatcccacgccc

SEQ ID NO: 659 - DNA, 17 bp, Artificial sequence
  Synthetic Oligonucleotide
taattcaatcccacgcc

SEQ ID NO: 660 - DNA, 17 bp, Artificial sequence
  Synthetic Oligonucleotide
ttaattcaatcccacgc

SEQ ID NO: 661 - DNA, 17 bp, Artificial sequence
  Synthetic Oligonucleotide
tttaattcaatcccacg

SEQ ID NO: 662 - DNA, 17 bp, Artificial sequence
  Synthetic Oligonucleotide
ttttaattcaatcccac

SEQ ID NO: 663 - DNA, 17 bp, Artificial sequence
  Synthetic Oligonucleotide
gttttaattcaatccca

SEQ ID NO: 664 - DNA, 17 bp, Artificial sequence
  Synthetic Oligonucleotide
tgttttaattcaatccc

SEQ ID NO: 665 - DNA, 17 bp, Artificial sequence
  Synthetic Oligonucleotide
ctgttttaattcaatcc

SEQ ID NO: 666 - DNA, 17 bp, Artificial sequence
  Synthetic Oligonucleotide
gctgttttaattcaatc

SEQ ID NO: 667 - DNA, 17 bp, Artificial sequence
  Synthetic Oligonucleotide
agctgttttaattcaat

SEQ ID NO: 668 - DNA, 17 bp, Artificial sequence
  Synthetic Oligonucleotide
cagctgttttaattcaa

SEQ ID NO: 669 - DNA, 17 bp, Artificial sequence
  Synthetic Oligonucleotide
gcagctgttttaattca

SEQ ID NO: 670 - DNA, 17 bp, Artificial sequence
  Synthetic Oligonucleotide
cgcagctgttttaattc

SEQ ID NO: 671 - DNA, 17 bp, Artificial sequence
  Synthetic Oligonucleotide
tcgcagctgttttaatt

SEQ ID NO: 672 - DNA, 17 bp, Artificial sequence
  Synthetic Oligonucleotide
gtcgcagctgttttaat

SEQ ID NO: 673 - DNA, 17 bp, Artificial sequence
  Synthetic Oligonucleotide
tgtcgcagctgttttaa

SEQ ID NO: 674 - DNA, 17 bp, Artificial sequence
  Synthetic Oligonucleotide
ttgtcgcagctgtttta

SEQ ID NO: 675 - DNA, 17 bp, Artificial sequence
  Synthetic Oligonucleotide
gttgtcgcagctgtttt

SEQ ID NO: 676 - DNA, 17 bp, Artificial sequence
  Synthetic Oligonucleotide
tgttgtcgcagctgttt

SEQ ID NO: 677 - DNA, 17 bp, Artificial sequence
  Synthetic Oligonucleotide
ttgttgtcgcagctgtt

SEQ ID NO: 678 - DNA, 17 bp, Artificial sequence
  Synthetic Oligonucleotide
tttgttgtcgcagctgt

SEQ ID NO: 679 - DNA, 17 bp, Artificial sequence
  Synthetic Oligonucleotide
ttttgttgtcgcagctg

SEQ ID NO: 680 - DNA, 17 bp, Artificial sequence
  Synthetic Oligonucleotide
tttttgttgtcgcagct

SEQ ID NO: 681 - DNA, 19 bp, Artificial sequence
  Synthetic Oligonucleotide
tagaaaacccaaatcctca

SEQ ID NO: 682 - DNA, 19 bp, Artificial sequence
  Synthetic Oligonucleotide
atagaaaacccaaatcctc

SEQ ID NO: 683 - DNA, 19 bp, Artificial sequence
  Synthetic Oligonucleotide
tatagaaaacccaaatcct

SEQ ID NO: 684 - DNA, 19 bp, Artificial sequence
  Synthetic Oligonucleotide
cttatagaaaacccaaatc

SEQ ID NO: 685 - DNA, 19 bp, Artificial sequence
  Synthetic Oligonucleotide
ccttatagaaaacccaaat

SEQ ID NO: 686 - DNA, 19 bp, Artificial sequence
  Synthetic Oligonucleotide
cccttatagaaaacccaaa

SEQ ID NO: 687 - DNA, 19 bp, Artificial sequence
  Synthetic Oligonucleotide
ccccttatagaaaacccaa

SEQ ID NO: 688 - DNA, 19 bp, Artificial sequence
  Synthetic Oligonucleotide
accccttatagaaaaccca

SEQ ID NO: 689 - DNA, 19 bp, Artificial sequence
  Synthetic Oligonucleotide
aaccccttatagaaaaccc

SEQ ID NO: 690 - DNA, 19 bp, Artificial sequence
  Synthetic Oligonucleotide
aaaccccttatagaaaacc

SEQ ID NO: 691 - DNA, 19 bp, Artificial sequence
  Synthetic Oligonucleotide
gaaaccccttatagaaaac

SEQ ID NO: 692 - DNA, 19 bp, Artificial sequence
  Synthetic Oligonucleotide
ggaaaccccttatagaaaa

SEQ ID NO: 693 - DNA, 19 bp, Artificial sequence
  Synthetic Oligonucleotide
aggaaaccccttatagaaa

SEQ ID NO: 694 - DNA, 19 bp, Artificial sequence
  Synthetic Oligonucleotide
caggaaaccccttatagaa

SEQ ID NO: 695 - DNA, 19 bp, Artificial sequence
  Synthetic Oligonucleotide
gcaggaaaccccttataga

SEQ ID NO: 696 - DNA, 19 bp, Artificial sequence
  Synthetic Oligonucleotide
agcaggaaaccccttatag

SEQ ID NO: 697 - DNA, 19 bp, Artificial sequence
  Synthetic Oligonucleotide
cagcaggaaaccccttata

SEQ ID NO: 698 - DNA, 19 bp, Artificial sequence
  Synthetic Oligonucleotide
ccagcaggaaaccccttat

SEQ ID NO: 699 - DNA, 19 bp, Artificial sequence
  Synthetic Oligonucleotide
tccagcaggaaacccctta

SEQ ID NO: 700 - DNA, 19 bp, Artificial sequence
  Synthetic Oligonucleotide
gtccagcaggaaacccctt

SEQ ID NO: 701 - DNA, 19 bp, Artificial sequence
  Synthetic Oligonucleotide
tgtccagcaggaaacccct

SEQ ID NO: 702 - DNA, 19 bp, Artificial sequence
  Synthetic Oligonucleotide
cctgtccagcaggaaaccc

SEQ ID NO: 703 - DNA, 19 bp, Artificial sequence
  Synthetic Oligonucleotide
ccctgtccagcaggaaacc

SEQ ID NO: 704 - DNA, 19 bp, Artificial sequence
  Synthetic Oligonucleotide
cccctgtccagcaggaaac

SEQ ID NO: 705 - DNA, 19 bp, Artificial sequence
  Synthetic Oligonucleotide
gcccctgtccagcaggaaa

SEQ ID NO: 706 - DNA, 19 bp, Artificial sequence
  Synthetic Oligonucleotide
acgcccctgtccagcagga

SEQ ID NO: 707 - DNA, 19 bp, Artificial sequence
  Synthetic Oligonucleotide
cacgcccctgtccagcagg

SEQ ID NO: 708 - DNA, 19 bp, Artificial sequence
  Synthetic Oligonucleotide
ccacgcccctgtccagcag

SEQ ID NO: 709 - DNA, 19 bp, Artificial sequence
  Synthetic Oligonucleotide
cccacgcccctgtccagca

SEQ ID NO: 710 - DNA, 19 bp, Artificial sequence
  Synthetic Oligonucleotide
tcccacgcccctgtccagc

SEQ ID NO: 711 - DNA, 19 bp, Artificial sequence
  Synthetic Oligonucleotide
atcccacgcccctgtccag

SEQ ID NO: 712 - DNA, 19 bp, Artificial sequence
  Synthetic Oligonucleotide
aatcccacgcccctgtcca

SEQ ID NO: 713 - DNA, 19 bp, Artificial sequence
  Synthetic Oligonucleotide
caatcccacgcccctgtcc

SEQ ID NO: 714 - DNA, 19 bp, Artificial sequence
  Synthetic Oligonucleotide
tcaatcccacgcccctgtc

SEQ ID NO: 715 - DNA, 19 bp, Artificial sequence
  Synthetic Oligonucleotide
ttcaatcccacgcccctgt

SEQ ID NO: 716 - DNA, 19 bp, Artificial sequence
  Synthetic Oligonucleotide
attcaatcccacgcccctg

SEQ ID NO: 717 - DNA, 19 bp, Artificial sequence
  Synthetic Oligonucleotide
aattcaatcccacgcccct

SEQ ID NO: 718 - DNA, 19 bp, Artificial sequence
  Synthetic Oligonucleotide
taattcaatcccacgcccc

SEQ ID NO: 719 - DNA, 19 bp, Artificial sequence
  Synthetic Oligonucleotide
ttaattcaatcccacgccc

SEQ ID NO: 720 - DNA, 19 bp, Artificial sequence
  Synthetic Oligonucleotide
tttaattcaatcccacgcc

SEQ ID NO: 721 - DNA, 19 bp, Artificial sequence
  Synthetic Oligonucleotide
ttttaattcaatcccacgc

SEQ ID NO: 722 - DNA, 19 bp, Artificial sequence
  Synthetic Oligonucleotide
gttttaattcaatcccacg

SEQ ID NO: 723 - DNA, 19 bp, Artificial sequence
  Synthetic Oligonucleotide
tgttttaattcaatcccac

SEQ ID NO: 724 - DNA, 19 bp, Artificial sequence
  Synthetic Oligonucleotide
ctgttttaattcaatccca

SEQ ID NO: 725 - DNA, 19 bp, Artificial sequence
  Synthetic Oligonucleotide
gctgttttaattcaatccc

SEQ ID NO: 726 - DNA, 19 bp, Artificial sequence
  Synthetic Oligonucleotide
agctgttttaattcaatcc

SEQ ID NO: 727 - DNA, 19 bp, Artificial sequence
  Synthetic Oligonucleotide
cagctgttttaattcaatc

SEQ ID NO: 728 - DNA, 19 bp, Artificial sequence
  Synthetic Oligonucleotide
gcagctgttttaattcaat

SEQ ID NO: 729 - DNA, 19 bp, Artificial sequence
  Synthetic Oligonucleotide
cgcagctgttttaattcaa

SEQ ID NO: 730 - DNA, 19 bp, Artificial sequence
  Synthetic Oligonucleotide
tcgcagctgttttaattca

SEQ ID NO: 731 - DNA, 19 bp, Artificial sequence
  Synthetic Oligonucleotide
gtcgcagctgttttaattc

SEQ ID NO: 732 - DNA, 19 bp, Artificial sequence
  Synthetic Oligonucleotide
tgtcgcagctgttttaatt

SEQ ID NO: 733 - DNA, 19 bp, Artificial sequence
  Synthetic Oligonucleotide
ttgtcgcagctgttttaat

SEQ ID NO: 734 - DNA, 19 bp, Artificial sequence
  Synthetic Oligonucleotide
gttgtcgcagctgttttaa

SEQ ID NO: 735 - DNA, 19 bp, Artificial sequence
  Synthetic Oligonucleotide
tgttgtcgcagctgtttta

SEQ ID NO: 736 - DNA, 19 bp, Artificial sequence
  Synthetic Oligonucleotide
ttgttgtcgcagctgtttt

SEQ ID NO: 737 - DNA, 19 bp, Artificial sequence
  Synthetic Oligonucleotide
tttgttgtcgcagctgttt

SEQ ID NO: 738 - DNA, 19 bp, Artificial sequence
  Synthetic Oligonucleotide
ttttgttgtcgcagctgtt

SEQ ID NO: 739 - DNA, 19 bp, Artificial sequence
  Synthetic Oligonucleotide
tttttgttgtcgcagctgt

SEQ ID NO: 740 - DNA, 18 bp, Artificial sequence
  Synthetic Oligonucleotide
ccccttatagaaaaccca

SEQ ID NO: 741 - DNA, 18 bp, Artificial sequence
  Synthetic Oligonucleotide
accccttatagaaaaccc

SEQ ID NO: 742 - DNA, 18 bp, Artificial sequence
  Synthetic Oligonucleotide
aaccccttatagaaaacc

SEQ ID NO: 743 - DNA, 18 bp, Artificial sequence
  Synthetic Oligonucleotide
aaaccccttatagaaaac

SEQ ID NO: 744 - DNA, 18 bp, Artificial sequence
  Synthetic Oligonucleotide
gaaaccccttatagaaaa

SEQ ID NO: 745 - DNA, 18 bp, Artificial sequence
  Synthetic Oligonucleotide
aggaaaccccttatagaa

SEQ ID NO: 746 - DNA, 18 bp, Artificial sequence
  Synthetic Oligonucleotide
caggaaaccccttataga

SEQ ID NO: 747 - DNA, 18 bp, Artificial sequence
  Synthetic Oligonucleotide
gcaggaaaccccttatag

SEQ ID NO: 748 - DNA, 18 bp, Artificial sequence
  Synthetic Oligonucleotide
agcaggaaaccccttata

SEQ ID NO: 749 - DNA, 18 bp, Artificial sequence
  Synthetic Oligonucleotide
cagcaggaaaccccttat

SEQ ID NO: 750 - DNA, 18 bp, Artificial sequence
  Synthetic Oligonucleotide
ccagcaggaaacccctta

SEQ ID NO: 751 - DNA, 18 bp, Artificial sequence
  Synthetic Oligonucleotide
tccagcaggaaacccctt

SEQ ID NO: 752 - DNA, 18 bp, Artificial sequence
  Synthetic Oligonucleotide
gtccagcaggaaacccct

SEQ ID NO: 753 - DNA, 18 bp, Artificial sequence
  Synthetic Oligonucleotide
tgtccagcaggaaacccc

SEQ ID NO: 754 - DNA, 18 bp, Artificial sequence
  Synthetic Oligonucleotide
ctgtccagcaggaaaccc

SEQ ID NO: 755 - DNA, 18 bp, Artificial sequence
  Synthetic Oligonucleotide
cctgtccagcaggaaacc

SEQ ID NO: 756 - DNA, 18 bp, Artificial sequence
  Synthetic Oligonucleotide
ccctgtccagcaggaaac

SEQ ID NO: 757 - DNA, 18 bp, Artificial sequence
  Synthetic Oligonucleotide
cccctgtccagcaggaaa

SEQ ID NO: 758 - DNA, 18 bp, Artificial sequence
  Synthetic Oligonucleotide
cgcccctgtccagcagga

SEQ ID NO: 759 - DNA, 18 bp, Artificial sequence
  Synthetic Oligonucleotide
acgcccctgtccagcagg

SEQ ID NO: 760 - DNA, 18 bp, Artificial sequence
  Synthetic Oligonucleotide
cacgcccctgtccagcag

SEQ ID NO: 761 - DNA, 18 bp, Artificial sequence
  Synthetic Oligonucleotide
ccacgcccctgtccagca

SEQ ID NO: 762 - DNA, 18 bp, Artificial sequence
  Synthetic Oligonucleotide
cccacgcccctgtccagc

SEQ ID NO: 763 - DNA, 18 bp, Artificial sequence
  Synthetic Oligonucleotide
tcccacgcccctgtccag

SEQ ID NO: 764 - DNA, 18 bp, Artificial sequence
  Synthetic Oligonucleotide
atcccacgcccctgtcca

SEQ ID NO: 765 - DNA, 18 bp, Artificial sequence
  Synthetic Oligonucleotide
aatcccacgcccctgtcc

SEQ ID NO: 766 - DNA, 18 bp, Artificial sequence
  Synthetic Oligonucleotide
caatcccacgcccctgtc

SEQ ID NO: 767 - DNA, 18 bp, Artificial sequence
  Synthetic Oligonucleotide
tcaatcccacgcccctgt

SEQ ID NO: 768 - DNA, 18 bp, Artificial sequence
  Synthetic Oligonucleotide
ttcaatcccacgcccctg

SEQ ID NO: 769 - DNA, 18 bp, Artificial sequence
  Synthetic Oligonucleotide
attcaatcccacgcccct

SEQ ID NO: 770 - DNA, 18 bp, Artificial sequence
  Synthetic Oligonucleotide
aattcaatcccacgcccc

SEQ ID NO: 771 - DNA, 18 bp, Artificial sequence
  Synthetic Oligonucleotide
taattcaatcccacgccc

SEQ ID NO: 772 - DNA, 18 bp, Artificial sequence
  Synthetic Oligonucleotide
ttaattcaatcccacgcc

SEQ ID NO: 773 - DNA, 18 bp, Artificial sequence
  Synthetic Oligonucleotide
tttaattcaatcccacgc

SEQ ID NO: 774 - DNA, 18 bp, Artificial sequence
  Synthetic Oligonucleotide
ttttaattcaatcccacg

SEQ ID NO: 775 - DNA, 18 bp, Artificial sequence
  Synthetic Oligonucleotide
gttttaattcaatcccac

SEQ ID NO: 776 - DNA, 18 bp, Artificial sequence
  Synthetic Oligonucleotide
tgttttaattcaatccca

SEQ ID NO: 777 - DNA, 18 bp, Artificial sequence
  Synthetic Oligonucleotide
ctgttttaattcaatccc

SEQ ID NO: 778 - DNA, 18 bp, Artificial sequence
  Synthetic Oligonucleotide
gctgttttaattcaatcc

SEQ ID NO: 779 - DNA, 18 bp, Artificial sequence
  Synthetic Oligonucleotide
agctgttttaattcaatc

SEQ ID NO: 780 - DNA, 18 bp, Artificial sequence
  Synthetic Oligonucleotide
cagctgttttaattcaat

SEQ ID NO: 781 - DNA, 18 bp, Artificial sequence
  Synthetic Oligonucleotide
gcagctgttttaattcaa

SEQ ID NO: 782 - DNA, 18 bp, Artificial sequence
  Synthetic Oligonucleotide
cgcagctgttttaattca

SEQ ID NO: 783 - DNA, 18 bp, Artificial sequence
  Synthetic Oligonucleotide
tcgcagctgttttaattc

SEQ ID NO: 784 - DNA, 18 bp, Artificial sequence
  Synthetic Oligonucleotide
gtcgcagctgttttaatt

SEQ ID NO: 785 - DNA, 18 bp, Artificial sequence
  Synthetic Oligonucleotide
tagaaaacccaaatcctc

SEQ ID NO: 786 - DNA, 18 bp, Artificial sequence
  Synthetic Oligonucleotide
atagaaaacccaaatcct

SEQ ID NO: 787 - DNA, 18 bp, Artificial sequence
  Synthetic Oligonucleotide
tatagaaaacccaaatcc

SEQ ID NO: 788 - DNA, 18 bp, Artificial sequence
  Synthetic Oligonucleotide
ttatagaaaacccaaatc

SEQ ID NO: 789 - DNA, 18 bp, Artificial sequence
  Synthetic Oligonucleotide
cttatagaaaacccaaat

SEQ ID NO: 790 - DNA, 18 bp, Artificial sequence
  Synthetic Oligonucleotide
ccttatagaaaacccaaa

SEQ ID NO: 791 - DNA, 18 bp, Artificial sequence
  Synthetic Oligonucleotide
cccttatagaaaacccaa

SEQ ID NO: 792 - DNA, 18 bp, Artificial sequence
  Synthetic Oligonucleotide
tgtcgcagctgttttaat

SEQ ID NO: 793 - DNA, 18 bp, Artificial sequence
  Synthetic Oligonucleotide
ttgtcgcagctgttttaa

SEQ ID NO: 794 - DNA, 18 bp, Artificial sequence
  Synthetic Oligonucleotide
gttgtcgcagctgtttta

SEQ ID NO: 795 - DNA, 18 bp, Artificial sequence
  Synthetic Oligonucleotide
tgttgtcgcagctgtttt

SEQ ID NO: 796 - DNA, 18 bp, Artificial sequence
  Synthetic Oligonucleotide
ttgttgtcgcagctgttt

SEQ ID NO: 797 - DNA, 18 bp, Artificial sequence
  Synthetic Oligonucleotide
tttgttgtcgcagctgtt

SEQ ID NO: 798 - DNA, 18 bp, Artificial sequence
  Synthetic Oligonucleotide
ttttgttgtcgcagctgt

SEQ ID NO: 799 - DNA, 18 bp, Artificial sequence
  Synthetic Oligonucleotide
tttttgttgtcgcagctg

SEQ ID NO: 800 - DNA, 16 bp, Artificial sequence
  Synthetic Oligonucleotide
aaaacccaaatcctca

SEQ ID NO: 801 - DNA, 16 bp, Artificial sequence
  Synthetic Oligonucleotide
agaaaacccaaatcct

SEQ ID NO: 802 - DNA, 16 bp, Artificial sequence
  Synthetic Oligonucleotide
tatagaaaacccaaat

SEQ ID NO: 803 - DNA, 16 bp, Artificial sequence
  Synthetic Oligonucleotide
ttatagaaaacccaaa

SEQ ID NO: 804 - DNA, 20 bp, Artificial sequence
  Synthetic Oligonucleotide
gcataagagggtaccagctg

SEQ ID NO: 805 - DNA, 20 bp, Artificial sequence
  Synthetic Oligonucleotide
gtcctttagccagggcagca

SEQ ID NO: 806 - DNA, 20 bp, Artificial sequence
  Synthetic Oligonucleotide
tccacccatgttgtgcaagc

SEQ ID NO: 807 - DNA, 20 bp, Artificial sequence
  Synthetic Oligonucleotide
ccacaccatgccacagagac

SEQ ID NO: 808 - DNA, 20 bp, Artificial sequence
  Synthetic Oligonucleotide
ttccgagtcaggctcttccc

SEQ ID NO: 809 - DNA, 20 bp, Artificial sequence
  Synthetic Oligonucleotide
ccttccctgaaggttcctcc

SEQ ID NO: 810 - DNA, 21 bp, Artificial sequence
  Primer
agtctctgtggcatggtttgg

SEQ ID NO: 811 - DNA, 21 bp, Artificial sequence
  primer
gggcgaatgactgagatcttg

SEQ ID NO: 812 - DNA, 27 bp, Artificial sequence
  Probe
taccgattaccacaagcaaccatggca

SEQ ID NO: 813 - DNA, 22 bp, Artificial sequence
  Primer
cgaagcagctcaatgaaatcaa

SEQ ID NO: 814 - DNA, 18 bp, Artificial sequence
  Primer
tgcctggagggccttctt

SEQ ID NO: 815 - DNA, 18 bp, Artificial sequence
  Probe
agaccacaagttgaagtc

SEQ ID NO: 816 - DNA, 20 bp, Artificial sequence
  Primer
gggcaaacagcaatttgtga

SEQ ID NO: 817 - DNA, 20 bp, Artificial sequence
  Primer
tggctacccaccttccttgt

SEQ ID NO: 818 - DNA, 28 bp, Artificial sequence
  Probe
ctggatactgtcccaatcccggtattcc

SEQ ID NO: 819 - DNA, 22 bp, Artificial sequence
  Synthetic Oligonucleotide
cgaagaagctcagtgaaatcaa

SEQ ID NO: 820 - DNA, 18 bp, Artificial sequence
  Synthetic Oligonucleotide
tgcctggagggccctctt

SEQ ID NO: 821 - DNA, 20 bp, Artificial sequence
  Synthetic Oligonucleotide
agcttcttgtccagctttat

SEQ ID NO: 822 - DNA, 21 bp, Artificial sequence
  Synthetic Oligonucleotide
agcttcttgtccagctttata

SEQ ID NO: 823 - DNA, 14 bp, Artificial sequence
  Synthetic Oligonucleotide
tcagtcatgacttc

SEQ ID NO: 824 - DNA, 15 bp, Artificial sequence
  Synthetic Oligonucleotide
tcagtcatgacttca

SEQ ID NO: 825 - DNA, 20 bp, Artificial sequence
  Synthetic Oligonucleotide
gctgattagagagaggtccc

SEQ ID NO: 826 - DNA, 20 bp, Artificial sequence
  Synthetic Oligonucleotide
tcccatttcaggagacctgg

SEQ ID NO: 827 - DNA, 15 bp, Artificial sequence
  Synthetic Oligonucleotide
atcagtcatgacttc

SEQ ID NO: 828 - DNA, 20 bp, Artificial sequence
  Synthetic Oligonucleotide
cggtgcaaggcttaggaatt

SEQ ID NO: 829 - DNA, 20 bp, Artificial sequence
  Synthetic Oligonucleotide
gcttcagtcatgacttcctt

SEQ ID NO: 830 - DNA, 21 bp, Artificial sequence
  Synthetic Oligonucleotide
gcttcagtcatgacttcctta

SEQ ID NO: 831 - DNA, 21 bp, Artificial sequence
  Synthetic Oligonucleotide
agcttcagtcatgacttcctt

SEQ ID NO: 832 - DNA, 20 bp, Artificial sequence
  Synthetic Oligonucleotide
tggtaatccactttcagagg

SEQ ID NO: 833 - DNA, 21 bp, Artificial sequence
  Synthetic Oligonucleotide
tggtaatccactttcagagga

SEQ ID NO: 834 - DNA, 21 bp, Artificial sequence
  Synthetic Oligonucleotide
tgcttcagtcatgacttcctt

SEQ ID NO: 835 - DNA, 20 bp, Artificial sequence
  Synthetic Oligonucleotide
cactgatttttgcccaggat

SEQ ID NO: 836 - DNA, 21 bp, Artificial sequence
  Synthetic Oligonucleotide
cactgatttttgcccaggata

SEQ ID NO: 837 - DNA, 21 bp, Artificial sequence
  Synthetic Oligonucleotide
aagcttcttgtccagctttat

SEQ ID NO: 838 - DNA, 20 bp, Artificial sequence
  Synthetic Oligonucleotide
acccaattcagaaggaagga

SEQ ID NO: 839 - DNA, 21 bp, Artificial sequence
  Synthetic Oligonucleotide
acccaattcagaaggaaggaa

SEQ ID NO: 840 - DNA, 21 bp, Artificial sequence
  Synthetic Oligonucleotide
aacccaattcagaaggaagga

SEQ ID NO: 841 - DNA, 21 bp, Artificial sequence
  Synthetic Oligonucleotide
atggtaatccactttcagagg

SEQ ID NO: 842 - DNA, 20 bp, Artificial sequence
  Synthetic Oligonucleotide
tcttggttacatgaaatccc

SEQ ID NO: 843 - DNA, 21 bp, Artificial sequence
  Synthetic Oligonucleotide
tcttggttacatgaaatccca

SEQ ID NO: 844 - DNA, 20 bp, Artificial sequence
  Synthetic Oligonucleotide
attcactttcataatgctgg

SEQ ID NO: 845 - DNA, 21 bp, Artificial sequence
  Synthetic Oligonucleotide
attcactttcataatgctgga

SEQ ID NO: 846 - DNA, 21 bp, Artificial sequence
  Synthetic Oligonucleotide
atcttggttacatgaaatccc

SEQ ID NO: 847 - DNA, 20 bp, Artificial sequence
  Synthetic Oligonucleotide
tgctccgttggtgcttgttc

SEQ ID NO: 848 - DNA, 20 bp, Artificial sequence
  Synthetic Oligonucleotide
atgcatggtgatgcttctga

SEQ ID NO: 849 - DNA, 20 bp, Artificial sequence
  Synthetic Oligonucleotide
cagctttattagggacagca

SEQ ID NO: 850 - DNA, 21 bp, Artificial sequence
  Synthetic Oligonucleotide
cagctttattagggacagcaa

SEQ ID NO: 851 - DNA, 21 bp, Artificial sequence
  Synthetic Oligonucleotide
acagctttattagggacagca

SEQ ID NO: 852 - DNA, 16 bp, Artificial sequence
  Synthetic Oligonucleotide
ttcagtcatgacttcc

SEQ ID NO: 853 - DNA, 20 bp, Artificial sequence
  Synthetic Oligonucleotide
  misc_feature (1)..(5): Bases at these positions are RNA
  misc_feature (16)..(20): Bases at these positions are RNA
gcuucagtcatgactuccuu

SEQ ID NO: 854 - DNA, 21 bp, Artificial sequence
  Synthetic Oligonucleotide
tgctccgttggtgcttgttca